European Patent Application EP 4 148 066 A1, published March 15, 2023. Title: T CELL ANTIGEN RECEPTOR, MULTIMERIC COMPLEX THEREOF, AND PREPARATION METHOD THEREFOR AND USE THEREOF. Applicant: CHINA IMMUNOTECH (BEIJING) BIOTECHNOLOGY CO., LTD、TSINGHUA UNIVERSITY. Application PCT/CN2021/089237. The sequence listing filed with the application follows.

SEQUENCE LISTING (366 sequences)

SEQ ID NO: 1 - protein, 294 aa, Artificial Sequence
  A0201-aa
MGSHSMRYFFTSVSRPGRGEPRFIAVGYVDDTQFVRFDSDAASQRMEPRAPWIEQEGPEYWDGETRKVKAHSQTHRVDLGTLRGYYNQSEAGSHTVQRMYGCDVGSDWRFLRGYHQYAYDGKDYIALKEDLRSWTAADMAAQTTKHKWEAAHVAEQLRAYLEGTCVEWLRRYLENGKETLQRTDAPKTHMTHHAVSDHEATLRCWALSFYPAEITLTWQRDGEDQTQDTELVETRPAGDGTFQKWVAVVVPSGQEQRYTCHVQHEGLPKPLTLRWEPGSGLNDIFEAQKIEWHE

SEQ ID NO: 2 - protein, 294 aa, Artificial Sequence
  A2402-aa
MGSHSMRYFSTSVSRPGRGEPRFIAVGYVDDTQFVRFDSDAASQRMEPRAPWIEQEGPEYWDEETGKVKAHSQTDRENLRIALRYYNQSEAGSHTLQMMFGCDVGSDGRFLRGYHQYAYDGKDYIALKEDLRSWTAADMAAQITKRKWEAAHVAEQQRAYLEGTCVDGLRRYLENGKETLQRTDPPKTHMTHHPISDHEATLRCWALGFYPAEITLTWQRDGEDQTQDTELVETRPAGDGTFQKWVAVVVPSGEEQRYTCHVQHEGLPKPLTLRWEPGSGLNDIFEAQKIEWHE

SEQ ID NO: 3 - protein, 294 aa, Artificial Sequence
  A1101-aa
MGSHSMRYFYTSVSRPGRGEPRFIAVGYVDDTQFVRFDSDAASQRMEPRAPWIEQEGPEYWDQETRNVKAQSQTDRVDLGTLRGYYNQSEDGSHTIQIMYGCDVGPDGRFLRGYRQDAYDGKDYIALNEDLRSWTAADMAAQITKRKWEAAHAAEQQRAYLEGRCVEWLRRYLENGKETLQRTDPPKTHMTHHPISDHEATLRCWALGFYPAEITLTWQRDGEDQTQDTELVETRPAGDGTFQKWVAVVVPSGEEQRYTCHVQHEGLPKPLTLRWELGSGLNDIFEAQKIEWHE

SEQ ID NO: 4 - protein, 101 aa, Artificial Sequence
  b2m-aa
MAIQRTPKIQVYSRHPAENGKSNFLNCYVSGFHPSDIEVDLLKNGERIEKVEHSDLSFSKDWSFYLLYYTEFTPTEKDEYACRVNHVTLSQPKIVKWDRDM

SEQ ID NO: 5 - protein, 609 aa, Artificial Sequence
  E23 aa
MSIGLLCCAALSLLWAGPVNAGVTQTPKFQVLKTGQSMTLQCAQDMNHEYMSWYRQDPGMGLRLIHYSVGAGITDQGEVPNGYNVSRSTTEDFPLRLLSAAPSQTSVYFCASSYQGGSSGYTFGSGTRLTVVEDLKNVFPPEVAVFEPSEAEISHTQKATLVCLATGFFPDHVELSWWVNGKEVHSGVSTDPQPLKEQPALNDSRYCLSSRLRVSATFWQNPRNHFRCQVQFYGLSENDEWTQDRAKPVTQIVSAEAWGRADCGFTSVSYQQGVLSATILYEILLGKATLYAVLVSALVLMAMVKRKDFRRKRSGSGATNFSLLKQAGDVEENPGPMETLLGVSLVILWLQLARVNSQQGEEDPQALSIQEGENATMNCSYKTSINNLQWYRQNSGRGLVHLILIRSNEREKHSGRLRVTLDTSKKSSSLLITASRAADTASYFCATEGDSGYSTLTFGKGTMLLVSPDIQNPDPAVYQLRDSKSSDKSVCLFTDFDSQTNVSQSKDSDVYITDKTVLDMRSMDFKSNSAVAWSNKSDFACANAFNNSIIPEDTFFPSPESSCDVKLVEKSFETDTNLNFQNLSVIGFRILLLKVAGFNLLMTLRLWSS

SEQ ID NO: 6 - protein, 609 aa, Artificial Sequence
  E240 aa
MSIGLLCCAALSLLWAGPVNAGVTQTPKFQVLKTGQSMTLQCAQDMNHEYMSWYRQDPGMGLRLIHYSVGAGITDQGEVPNGYNVSRSTTEDFPLRLLSAAPSQTSVYFCASSGQGGGYGYTFGSGTRLTVVEDLKNVFPPEVAVFEPSEAEISHTQKATLVCLATGFFPDHVELSWWVNGKEVHSGVSTDPQPLKEQPALNDSRYCLSSRLRVSATFWQNPRNHFRCQVQFYGLSENDEWTQDRAKPVTQIVSAEAWGRADCGFTSVSYQQGVLSATILYEILLGKATLYAVLVSALVLMAMVKRKDFRRKRSGSGATNFSLLKQAGDVEENPGPMETLLGVSLVILWLQLARVNSQQGEEDPQALSIQEGENATMNCSYKTSINNLQWYRQNSGRGLVHLILIRSNEREKHSGRLRVTLDTSKKSSSLLITASRAADTASYFCATVGDSGYSTLTFGKGTMLLVSPDIQNPDPAVYQLRDSKSSDKSVCLFTDFDSQTNVSQSKDSDVYITDKTVLDMRSMDFKSNSAVAWSNKSDFACANAFNNSIIPEDTFFPSPESSCDVKLVEKSFETDTNLNFQNLSVIGFRILLLKVAGFNLLMTLRLWSS

SEQ ID NO: 7 - protein, 613 aa, Artificial Sequence
  E29 aa
MLLLLLLLGPGSGLGAVVSQHPSRVICKSGTSVKIECRSLDFQATTMFWYRQFPKKSLMLMATSNEGSKATYEQGVEKDKFLINHASLTLSTLTVTSAHPEDSSFYICSARDTSGVNFYNEQFFGPGTRLTVLEDLKNVFPPEVAVFEPSEAEISHTQKATLVCLATGFFPDHVELSWWVNGKEVHSGVSTDPQPLKEQPALNDSRYCLSSRLRVSATFWQNPRNHFRCQVQFYGLSENDEWTQDRAKPVTQIVSAEAWGRADCGFTSVSYQQGVLSATILYEILLGKATLYAVLVSALVLMAMVKRKDFRRKRSGSGATNFSLLKQAGDVEENPGPMEKNPLAAPLLILWFHLDCVSSILNVEQSPQSLHVQEGDSTNFTCSFPSSNFYALHWYRWETAKSPEALFVMTLNGDEKKKGRISATLNTKEGYSYLYIKGSQPEDSATYLCASTNSNSGYALNFGKGTSLLVTPHIQNPDPAVYQLRDSKSSDKSVCLFTDFDSQTNVSQSKDSDVYITDKTVLDMRSMDFKSNSAVAWSNKSDFACANAFNNSIIPEDTFFPSPESSCDVKLVEKSFETDTNLNFQNLSVIGFRILLLKVAGFNLLMTLRLWSS

SEQ ID NO: 8 - protein, 607 aa, Artificial Sequence
  E180-1 aa
MSNQVLCCVVLCFLGANTVDGGITQSPKYLFRKEGQNVTLSCEQNLNHDAMYWYRQDPGQGLRLIYYSQIVNDFQKGDIAEGYSVSREKKESFPLTVTSAQKNPTAFYLCASAITGGTEAFFGQGTRLTVVEDLKNVFPPEVAVFEPSEAEISHTQKATLVCLATGFFPDHVELSWWVNGKEVHSGVSTDPQPLKEQPALNDSRYCLSSRLRVSATFWQNPRNHFRCQVQFYGLSENDEWTQDRAKPVTQIVSAEAWGRADCGFTSVSYQQGVLSATILYEILLGKATLYAVLVSALVLMAMVKRKDFRRKRSGSGATNFSLLKQAGDVEENPGPMTSIRAVFIFLWLQLDLVNGENVEQHPSTLSVQEGDSAVIKCTYSDSASNYFPWYKQELGKGPQLIIDIRSNVGEKKDQRIAVTLNKTAKHFSLHITETQPEDSAVYFCAARGGGYSTLTFGKGTMLLVSPDIQNPDPAVYQLRDSKSSDKSVCLFTDFDSQTNVSQSKDSDVYITDKTVLDMRSMDFKSNSAVAWSNKSDFACANAFNNSIIPEDTFFPSPESSCDVKLVEKSFETDTNLNFQNLSVIGFRILLLKVAGFNLLMTLRLWSS

SEQ ID NO: 9 - protein, 614 aa, Artificial Sequence
  E44 aa
MGPQLLGYVVLCLLGAGPLEAQVTQNPRYLITVTGKKLTVTCSQNMNHEYMSWYRQDPGLGLRQIYYSMNVEVTDKGDVPEGYKVSRKEKRNFPLILESPSPNQTSLYFCASTPLPTSSGRLGEQYFGPGTRLTVTEDLKNVFPPEVAVFEPSEAEISHTQKATLVCLATGFFPDHVELSWWVNGKEVHSGVSTDPQPLKEQPALNDSRYCLSSRLRVSATFWQNPRNHFRCQVQFYGLSENDEWTQDRAKPVTQIVSAEAWGRADCGFTSVSYQQGVLSATILYEILLGKATLYAVLVSALVLMAMVKRKDFRRKRSGSGATNFSLLKQAGDVEENPGPMMKSLRVLLVILWLQLSWVWSQQKEVEQDPGPLSVPEGAIVSLNCTYSNSAFQYFMWYRQYSRKGPELLMYTYSSGNKEDGRFTAQVDKSSKYISLFIRDSQPSDSATYLCAMFRSTLGRLYFGRGTQLTVWPDIQNPDPAVYQLRDSKSSDKSVCLFTDFDSQTNVSQSKDSDVYITDKTVLDMRSMDFKSNSAVAWSNKSDFACANAFNNSIIPEDTFFPSPESSCDVKLVEKSFETDTNLNFQNLSVIGFRILLLKVAGFNLLMTLRLWSS

SEQ ID NO: 10 - protein, 603 aa, Artificial Sequence
  E141 aa
MGCRLLCCAVLCLLGAVPIDTEVTQTPKHLVMGMTNKKSLKCEQHMGHRAMYWYKQKAKKPPELMFVYSYEKLSINESVPSRFSPECPNSSLLNLHLHALQPEDSALYLCASSQGRWYEQYFGPGTRLTVTEDLKNVFPPEVAVFEPSEAEISHTQKATLVCLATGFFPDHVELSWWVNGKEVHSGVSTDPQPLKEQPALNDSRYCLSSRLRVSATFWQNPRNHFRCQVQFYGLSENDEWTQDRAKPVTQIVSAEAWGRADCGFTSVSYQQGVLSATILYEILLGKATLYAVLVSALVLMAMVKRKDFRRKRSGSGATNFSLLKQAGDVEENPGPMKRILGALLGLLSAQVCCVRGIQVEQSPPDLILQEGANSTLRCNFSDSVNNLQWFHQNPWGQLINLFYIPSGTKQNGRLSATTVATERYSLLYISSSQTTDSGVYFCAVLNNNDMRFGAGTRLTVKPNIQNPDPAVYQLRDSKSSDKSVCLFTDFDSQTNVSQSKDSDVYITDKTVLDMRSMDFKSNSAVAWSNKSDFACANAFNNSIIPEDTFFPSPESSCDVKLVEKSFETDTNLNFQNLSVIGFRILLLKVAGFNLLMTLRLWSS

SEQ ID NO: 11 - protein, 603 aa, Artificial Sequence
  E149 aa
MGCRLLCCAVLCLLGAVPIDTEVTQTPKHLVMGMTNKKSLKCEQHMGHRAMYWYKQKAKKPPELMFVYSYEKLSINESVPSRFSPECPNSSLLNLHLHALQPEDSALYLCASSPGRWYEQFFGPGTRLTVLEDLKNVFPPEVAVFEPSEAEISHTQKATLVCLATGFFPDHVELSWWVNGKEVHSGVSTDPQPLKEQPALNDSRYCLSSRLRVSATFWQNPRNHFRCQVQFYGLSENDEWTQDRAKPVTQIVSAEAWGRADCGFTSVSYQQGVLSATILYEILLGKATLYAVLVSALVLMAMVKRKDFRRKRSGSGATNFSLLKQAGDVEENPGPMKRILGALLGLLSAQVCCVRGIQVEQSPPDLILQEGANSTLRCNFSDSVNNLQWFHQNPWGQLINLFYIPSGTKQNGRLSATTVATERYSLLYISSSQTTDSGVYFCAVVDNNDMRFGAGTRLTVKPNIQNPDPAVYQLRDSKSSDKSVCLFTDFDSQTNVSQSKDSDVYITDKTVLDMRSMDFKSNSAVAWSNKSDFACANAFNNSIIPEDTFFPSPESSCDVKLVEKSFETDTNLNFQNLSVIGFRILLLKVAGFNLLMTLRLWSS

SEQ ID NO: 12 - protein, 608 aa, Artificial Sequence
  E168 aa
MGPGLLCWVLLCLLGAGPVDAGVTQSPTHLIKTRGQHVTLRCSPISGHKSVSWYQQVLGQGPQFIFQYYEKEERGRGNFPDRFSARQFPNYSSELNVNALLLGDSALYLCASSLDRDRNDYGYTFGSGTRLTVVEDLKNVFPPEVAVFEPSEAEISHTQKATLVCLATGFFPDHVELSWWVNGKEVHSGVSTDPQPLKEQPALNDSRYCLSSRLRVSATFWQNPRNHFRCQVQFYGLSENDEWTQDRAKPVTQIVSAEAWGRADCGFTSVSYQQGVLSATILYEILLGKATLYAVLVSALVLMAMVKRKDFRRKRSGSGATNFSLLKQAGDVEENPGPMKKLLAMILWLQLDRLSGELKVEQNPLFLSMQEGKNYTIYCNYSTTSDRLYWYRQDPGKSLESLFVLLSNGAVKQEGRLMASLDTKARLSTLHITAAVHDLSATYFCAVAMNRDDKIIFGKGTRLHILPNIQNPDPAVYQLRDSKSSDKSVCLFTDFDSQTNVSQSKDSDVYITDKTVLDMRSMDFKSNSAVAWSNKSDFACANAFNNSIIPEDTFFPSPESSCDVKLVEKSFETDTNLNFQNLSVIGFRILLLKVAGFNLLMTLRLWSS

SEQ ID NO: 13 - protein, 615 aa, Artificial Sequence
  E170 aa
MDTRVLCCAVICLLGAGLSNAGVMQNPRHLVRRRGQEARLRCSPMKGHSHVYWYRQLPEEGLKFMVYLQKENIIDESGMPKERFSAEFPKEGPSILRIQQVVRGDSAAYFCASSPAPRAGNQPQHFGDGTRLSILEDLKNVFPPEVAVFEPSEAEISHTQKATLVCLATGFFPDHVELSWWVNGKEVHSGVSTDPQPLKEQPALNDSRYCLSSRLRVSATFWQNPRNHFRCQVQFYGLSENDEWTQDRAKPVTQIVSAEAWGRADCGFTSVSYQQGVLSATILYEILLGKATLYAVLVSALVLMAMVKRKDFRRKRSGSGATNFSLLKQAGDVEENPGPMTSIRAVFIFLWLQLDLVNGENVEQHPSTLSVQEGDSAVIKCTYSDSASNYFPWYKQELGKRPQLIIDIRSNVGEKKDQRIAVTLNKTAKHFSLHITETQPEDSAVYFCAAREGFYQTGANNLFFGTGTRLTVIPYIQNPDPAVYQLRDSKSSDKSVCLFTDFDSQTNVSQSKDSDVYITDKTVLDMRSMDFKSNSAVAWSNKSDFACANAFNNSIIPEDTFFPSPESSCDVKLVEKSFETDTNLNFQNLSVIGFRILLLKVAGFNLLMTLRLWSS

SEQ ID NO: 14 - protein, 612 aa, Artificial Sequence
  E244/303 aa
MGPQLLGYVVLCLLGAGPLEAQVTQNPRYLITVTGKKLTVTCSQNMNHEYMSWYRQDPGLGLRQIYYSMNVEVTDKGDVPEGYKVSRKEKRNFPLILESPSPNQTSLYFCASSLYPPGHSNQPQHFGDGTRLSILEDLKNVFPPEVAVFEPSEAEISHTQKATLVCLATGFFPDHVELSWWVNGKEVHSGVSTDPQPLKEQPALNDSRYCLSSRLRVSATFWQNPRNHFRCQVQFYGLSENDEWTQDRAKPVTQIVSAEAWGRADCGFTSVSYQQGVLSATILYEILLGKATLYAVLVSALVLMAMVKRKDFRRKRSGSGATNFSLLKQAGDVEENPGPMTSIRAVFIFLWLQLDLVNGENVEQHPSTLSVQEGDSAVIKCTYSDSASNYFPWYKQELGKRPQLIIDIRSNVGEKKDQRIAVTLNKTAKHFSLHITETQPEDSAVYFCAATAGGATNKLIFGTGTLLAVQPNIQNPDPAVYQLRDSKSSDKSVCLFTDFDSQTNVSQSKDSDVYITDKTVLDMRSMDFKSNSAVAWSNKSDFACANAFNNSIIPEDTFFPSPESSCDVKLVEKSFETDTNLNFQNLSVIGFRILLLKVAGFNLLMTLRLWSS

SEQ ID NO: 15 - protein, 606 aa, Artificial Sequence
  E245 aa
MGPGLLCWVLLCLLGAGPVDAGVTQSPTHLIKTRGQHVTLRCSPISGHKSVSWYQQVLGQGPQFIFQYYEKEERGRGNFPDRFSARQFPNYSSELNVNALLLGDSALYLCASSLEPGWGDTQYFGPGTRLTVLEDLKNVFPPEVAVFEPSEAEISHTQKATLVCLATGFFPDHVELSWWVNGKEVHSGVSTDPQPLKEQPALNDSRYCLSSRLRVSATFWQNPRNHFRCQVQFYGLSENDEWTQDRAKPVTQIVSAEAWGRADCGFTSVSYQQGVLSATILYEILLGKATLYAVLVSALVLMAMVKRKDFRRKRSGSGATNFSLLKQAGDVEENPGPMKKLLAMILWLQLDRLSGELKVEQNPLFLSMQEGKNYTIYCNYSTTSDRLYWYRQDPGKSLESLFVLLSNGAVKQEGRLMASLDTKARLSTLHITAAVHDLSATYFCAVELTGNQFYFGTGTSLTVIPNIQNPDPAVYQLRDSKSSDKSVCLFTDFDSQTNVSQSKDSDVYITDKTVLDMRSMDFKSNSAVAWSNKSDFACANAFNNSIIPEDTFFPSPESSCDVKLVEKSFETDTNLNFQNLSVIGFRILLLKVAGFNLLMTLRLWSS

SEQ ID NO: 16 - protein, 603 aa, Artificial Sequence
  E254 aa
MGFRLLCCVAFCLLGAGPVDSGVTQTPKHLITATGQRVTLRCSPRSGDLSVYWYQQSLDQGLQFLIQYYNGEERAKGNILERFSAQQFPDLHSELNLSSLELGDSALYFCASSVGPWYEQYFGPGTRLTVTEDLKNVFPPEVAVFEPSEAEISHTQKATLVCLATGFFPDHVELSWWVNGKEVHSGVSTDPQPLKEQPALNDSRYCLSSRLRVSATFWQNPRNHFRCQVQFYGLSENDEWTQDRAKPVTQIVSAEAWGRADCGFTSVSYQQGVLSATILYEILLGKATLYAVLVSALVLMAMVKRKDFRRKRSGSGATNFSLLKQAGDVEENPGPMKRILGALLGLLSAQVCCVRGIQVEQSPPDLILQEGANSTLRCNFSDSVNNLQWFHQNPWGQLINLFYIPSGTKQNGRLSATTVATERYSLLYISSSQTTDSGVYFCAVLNNNDMRFGAGTRLTVKPNIQNPDPAVYQLRDSKSSDKSVCLFTDFDSQTNVSQSKDSDVYITDKTVLDMRSMDFKSNSAVAWSNKSDFACANAFNNSIIPEDTFFPSPESSCDVKLVEKSFETDTNLNFQNLSVIGFRILLLKVAGFNLLMTLRLWSS

SEQ ID NO: 17 - protein, 603 aa, Artificial Sequence
  E301aa
MGCRLLCCAVLCLLGAVPIDTEVTQTPKHLVMGMTNKKSLKCEQHMGHRAMYWYKQKAKKPPELMFVYSYEKLSINESVPSRFSPECPNSSLLNLHLHALQPEDSALYLCASSPGRFYEQYFGPGTRLTVTEDLKNVFPPEVAVFEPSEAEISHTQKATLVCLATGFFPDHVELSWWVNGKEVHSGVSTDPQPLKEQPALNDSRYCLSSRLRVSATFWQNPRNHFRCQVQFYGLSENDEWTQDRAKPVTQIVSAEAWGRADCGFTSVSYQQGVLSATILYEILLGKATLYAVLVSALVLMAMVKRKDFRRKRSGSGATNFSLLKQAGDVEENPGPMKRILGALLGLLSAQVCCVRGIQVEQSPPDLILQEGANSTLRCNFSDSVNNLQWFHQNPWGQLINLFYIPSGTKQNGRLSATTVATERYSLLYISSSQTTDSGVYFCAVLNNNDMRFGAGTRLTVKPNIQNPDPAVYQLRDSKSSDKSVCLFTDFDSQTNVSQSKDSDVYITDKTVLDMRSMDFKSNSAVAWSNKSDFACANAFNNSIIPEDTFFPSPESSCDVKLVEKSFETDTNLNFQNLSVIGFRILLLKVAGFNLLMTLRLWSS

SEQ ID NO: 18 - protein, 603 aa, Artificial Sequence
  E304 aa
MGCRLLCCAVLCLLGAVPIDTEVTQTPKHLVMGMTNKKSLKCEQHMGHRAMYWYKQKAKKPPELMFVYSYEKLSINESVPSRFSPECPNSSLLNLHLHALQPEDSALYLCASSPGRWYEQYFGPGTRLTVTEDLKNVFPPEVAVFEPSEAEISHTQKATLVCLATGFFPDHVELSWWVNGKEVHSGVSTDPQPLKEQPALNDSRYCLSSRLRVSATFWQNPRNHFRCQVQFYGLSENDEWTQDRAKPVTQIVSAEAWGRADCGFTSVSYQQGVLSATILYEILLGKATLYAVLVSALVLMAMVKRKDFRRKRSGSGATNFSLLKQAGDVEENPGPMKRILGALLGLLSAQVCCVRGIQVEQSPPDLILQEGANSTLRCNFSDSVNNLQWFHQNPWGQLINLFYIPSGTKQNGRLSATTVATERYSLLYISSSQTTDSGVYFCAVVDNNDMRFGAGTRLTVKPNIQNPDPAVYQLRDSKSSDKSVCLFTDFDSQTNVSQSKDSDVYITDKTVLDMRSMDFKSNSAVAWSNKSDFACANAFNNSIIPEDTFFPSPESSCDVKLVEKSFETDTNLNFQNLSVIGFRILLLKVAGFNLLMTLRLWSS

SEQ ID NO: 19 - protein, 608 aa, Artificial Sequence
  E305 aa
MDTWLVCWAIFSLLKAGLTEPEVTQTPSHQVTQMGQEVILRCVPISNHLYFYWYRQILGQKVEFLVSFYNNEISEKSEIFDDQFSVERPDGSNFTLKIRSTKLEDSAMYFCASSEGPTGTSYEQYFGPGTRLTVTEDLKNVFPPEVAVFEPSEAEISHTQKATLVCLATGFFPDHVELSWWVNGKEVHSGVSTDPQPLKEQPALNDSRYCLSSRLRVSATFWQNPRNHFRCQVQFYGLSENDEWTQDRAKPVTQIVSAEAWGRADCGFTSVSYQQGVLSATILYEILLGKATLYAVLVSALVLMAMVKRKDFRRKRSGSGATNFSLLKQAGDVEENPGPMKKLLAMILWLQLDRLSGELKVEQNPLFLSMQEGKNYTIYCNYSTTSDRLYWYRQDPGKSLESLFVLLSNGAVKQEGRLMASLDTKARLSTLHITAAVHDLSATYFCAVNTGFQKLVFGTGTRLLVSPNIQNPDPAVYQLRDSKSSDKSVCLFTDFDSQTNVSQSKDSDVYITDKTVLDMRSMDFKSNSAVAWSNKSDFACANAFNNSIIPEDTFFPSPESSCDVKLVEKSFETDTNLNFQNLSVIGFRILLLKVAGFNLLMTLRLWSS

SEQ ID NO: 20 - protein, 615 aa, Artificial Sequence
  E307 aa
MGTRLLCWVVLGFLGTDHTGAGVSQSPRYKVAKRGQDVALRCDPISGHVSLFWYQQALGQGPEFLTYFQNEAQLDKSGLPSDRFFAERPEGSVSTLKIQRTQQEDSAVYLCASSQESGGTDTQYFGPGTRLTVLEDLKNVFPPEVAVFEPSEAEISHTQKATLVCLATGFFPDHVELSWWVNGKEVHSGVSTDPQPLKEQPALNDSRYCLSSRLRVSATFWQNPRNHFRCQVQFYGLSENDEWTQDRAKPVTQIVSAEAWGRADCGFTSVSYQQGVLSATILYEILLGKATLYAVLVSALVLMAMVKRKDFRRKRSGSGATNFSLLKQAGDVEENPGPMLTASLLRAVIASICVVSSMAQKVTQAQTEISVVEKEDVTLDCVYETRDTTYYLFWYKQPPSGELVFLIRRNSFDEQNEISGRYSWNFQKSTSSFNFTITASQVVDSAVYFCALSEPPSGTYKYIFGTGTRLKVLANIQNPDPAVYQLRDSKSSDKSVCLFTDFDSQTNVSQSKDSDVYITDKTVLDMRSMDFKSNSAVAWSNKSDFACANAFNNSIIPEDTFFPSPESSCDVKLVEKSFETDTNLNFQNLSVIGFRILLLKVAGFNLLMTLRLWSS

SEQ ID NO: 21 - protein, 603 aa, Artificial Sequence
  E314 aa
MGCRLLCCAVLCLLGAVPIDTEVTQTPKHLVMGMTNKKSLKCEQHMGHRAMYWYKQKAKKPPELMFVYSYEKLSINESVPSRFSPECPNSSLLNLHLHALQPEDSALYLCASSQGRWYEQYFGPGTRLTVTEDLKNVFPPEVAVFEPSEAEISHTQKATLVCLATGFFPDHVELSWWVNGKEVHSGVSTDPQPLKEQPALNDSRYCLSSRLRVSATFWQNPRNHFRCQVQFYGLSENDEWTQDRAKPVTQIVSAEAWGRADCGFTSVSYQQGVLSATILYEILLGKATLYAVLVSALVLMAMVKRKDFRRKRSGSGATNFSLLKQAGDVEENPGPMKRILGALLGLLSAQVCCVRGIQVEQSPPDLILQEGANSTLRCNFSDSVNNLQWFHQNPWGQLINLFYIPSGTKQNGRLSATTVATERYSLLYISSSQTTDSGVYFCAVLDNNDMRFGAGTRLTVKPNIQNPDPAVYQLRDSKSSDKSVCLFTDFDSQTNVSQSKDSDVYITDKTVLDMRSMDFKSNSAVAWSNKSDFACANAFNNSIIPEDTFFPSPESSCDVKLVEKSFETDTNLNFQNLSVIGFRILLLKVAGFNLLMTLRLWSS

SEQ ID NO: 22 - protein, 608 aa, Artificial Sequence
  E315 aa
MGTRLLCWAALCLLGAELTEAGVAQSPRYKIIEKRQSVAFWCNPISGHATLYWYQQILGQGPKLLIQFQNNGVVDDSQLPKDRFSAERLKGVDSTLKIQPAKLEDSAVYLCASSVFPTSVEQYFGPGTRLTVTEDLKNVFPPEVAVFEPSEAEISHTQKATLVCLATGFFPDHVELSWWVNGKEVHSGVSTDPQPLKEQPALNDSRYCLSSRLRVSATFWQNPRNHFRCQVQFYGLSENDEWTQDRAKPVTQIVSAEAWGRADCGFTSVSYQQGVLSATILYEILLGKATLYAVLVSALVLMAMVKRKDFRRKRSGSGATNFSLLKQAGDVEENPGPMETLLGLLILWLQLQWVSSKQEVTQIPAALSVPEGENLVLNCSFTDSAIYNLQWFRQDPGKGLTSLLLIQSSQREQTSGRLNASLDKSSGRSTLYIAASQPGDSATYLCAGKTSYDKVIFGPGTSLSVIPNIQNPDPAVYQLRDSKSSDKSVCLFTDFDSQTNVSQSKDSDVYITDKTVLDMRSMDFKSNSAVAWSNKSDFACANAFNNSIIPEDTFFPSPESSCDVKLVEKSFETDTNLNFQNLSVIGFRILLLKVAGFNLLMTLRLWSS

SEQ ID NO: 23 - protein, 616 aa, Artificial Sequence
  E316 aa
MSNQVLCCVVLCLLGANTVDGGITQSPKYLFRKEGQNVTLSCEQNLNHDAMYWYRQDPGQGLRLIYYSQIVNDFQKGDIAEGYSVSREKKESFPLTVTSAQKNPTAFYLCASSIGVGLSNTEAFFGQGTRLTVVEDLKNVFPPEVAVFEPSEAEISHTQKATLVCLATGFFPDHVELSWWVNGKEVHSGVSTDPQPLKEQPALNDSRYCLSSRLRVSATFWQNPRNHFRCQVQFYGLSENDEWTQDRAKPVTQIVSAEAWGRADCGFTSVSYQQGVLSATILYEILLGKATLYAVLVSALVLMAMVKRKDFRRKRSGSGATNFSLLKQAGDVEENPGPMSLSSLLKVVTASLWLGPGIAQKITQTQPGMFVQEKEAVTLDCTYDTSDQSYGLFWYKQPSSGEMIFLIYQGSYDEQNATEGRYSLNFQKARKSANLVISASQLGDSAMYFCAMVSGAGGGADGLTFGKGTHLIIQPYIQNPDPAVYQLRDSKSSDKSVCLFTDFDSQTNVSQSKDSDVYITDKTVLDMRSMDFKSNSAVAWSNKSDFACANAFNNSIIPEDTFFPSPESSCDVKLVEKSFETDTNLNFQNLSVIGFRILLLKVAGFNLLMTLRLWSS

SEQ ID NO: 24 - protein, 609 aa, Artificial Sequence
  E317 aa
MGPQLLGYVVLCLLGAGPLEAQVTQNPRYLITVTGKKLTVTCSQNMNHEYMSWYRQDPGLGLRQIYYSMNVEVTDKGDVPEGYKVSRKEKRNFPLILESPSPNQTSLYFCASSLWTSNSPLHFGNGTRLTVTEDLKNVFPPEVAVFEPSEAEISHTQKATLVCLATGFFPDHVELSWWVNGKEVHSGVSTDPQPLKEQPALNDSRYCLSSRLRVSATFWQNPRNHFRCQVQFYGLSENDEWTQDRAKPVTQIVSAEAWGRADCGFTSVSYQQGVLSATILYEILLGKATLYAVLVSALVLMAMVKRKDFRRKRSGSGATNFSLLKQAGDVEENPGPMAGIRALFMYLWLQLDWVSRGESVGLHLPTLSVQEGDNSIINCAYSNSASDYFIWYKQESGKGPQFIIDIRSNMDKRQGQRVTVLLNKTVKHLSLQIAATQPGDSAVYFCAETPGGYQKVTFGTGTKLQVIPNIQNPDPAVYQLRDSKSSDKSVCLFTDFDSQTNVSQSKDSDVYITDKTVLDMRSMDFKSNSAVAWSNKSDFACANAFNNSIIPEDTFFPSPESSCDVKLVEKSFETDTNLNFQNLSVIGFRILLLKVAGFNLLMTLRLWSS

SEQ ID NO: 25 - protein, 609 aa, Artificial Sequence
  E318 aa
MDSWTFCCVSLCILVAKHTDAGVIQSPRHEVTEMGQEVTLRCKPISGHNSLFWYRQTMMRGLELLIYFNNNVPIDDSGMPEDRFSAKMPNASFSTLKIQPSEPRDSAVYFCASSLGAGHLWGYTFGSGTRLTVVEDLKNVFPPEVAVFEPSEAEISHTQKATLVCLATGFFPDHVELSWWVNGKEVHSGVSTDPQPLKEQPALNDSRYCLSSRLRVSATFWQNPRNHFRCQVQFYGLSENDEWTQDRAKPVTQIVSAEAWGRADCGFTSVSYQQGVLSATILYEILLGKATLYAVLVSALVLMAMVKRKDFRRKRSGSGATNFSLLKQAGDVEENPGPMTSIRAVFIFLWLQLDLVNGENVEQHPSTLSVQEGDSAVIKCTYSDSASNYFPWYKQELGKRPQLIIDIRSNVGEKKDQRIAVTLNKTAKHFSLHITETQPEDSAVYFCAASNRDDKIIFGKGTRLHILPNIQNPDPAVYQLRDSKSSDKSVCLFTDFDSQTNVSQSKDSDVYITDKTVLDMRSMDFKSNSAVAWSNKSDFACANAFNNSIIPEDTFFPSPESSCDVKLVEKSFETDTNLNFQNLSVIGFRILLLKVAGFNLLMTLRLWSS

SEQ ID NO: 26 - protein, 609 aa, Artificial Sequence
  E320 aa
MGTRLLCWVVLGFLGTDHTGAGVSQSPRYKVAKRGQDVALRCDPISGHVSLFWYQQALGQGPEFLTYFQNEAQLDKSGLPSDRFFAERPEGSVSTLKIQRTQQEDSAVYLCASREGVGLYEQYFGPGTRLTVTEDLKNVFPPEVAVFEPSEAEISHTQKATLVCLATGFFPDHVELSWWVNGKEVHSGVSTDPQPLKEQPALNDSRYCLSSRLRVSATFWQNPRNHFRCQVQFYGLSENDEWTQDRAKPVTQIVSAEAWGRADCGFTSVSYQQGVLSATILYEILLGKATLYAVLVSALVLMAMVKRKDFRRKRSGSGATNFSLLKQAGDVEENPGPMKKLLAMILWLQLDRLSGELKVEQNPLFLSMQEGKNYTIYCNYSTTSDRLYWYRQDPGKSLESLFVLLSNGAVKQEGRLMASLDTKARLSTLHITAAVHDLSATYFCAVDIGTEYGNKLVFGAGTILRVKSYIQNPDPAVYQLRDSKSSDKSVCLFTDFDSQTNVSQSKDSDVYITDKTVLDMRSMDFKSNSAVAWSNKSDFACANAFNNSIIPEDTFFPSPESSCDVKLVEKSFETDTNLNFQNLSVIGFRILLLKVAGFNLLMTLRLWSS

SEQ ID NO: 27 - protein, 497 aa, Artificial Sequence
  LMP2 aa
MGSLEMVPMGAGPPSPGGDPDGYDGGNNSQYPSASGSSGNTPTPPNDEERESNEEPPPPYEDPYWGNGDRHSDYQPLGTQDQSLYLGLQHDGNDGLPPPPYSPRDDSSQHIYEEAGRGSMNPVCLPVIVAPYLFWLAAIAASCFTASVSTVVTATGLALSLLLLAAVASSYAAAQRKLLTPVTVLTAVVTFFAICLTWRIEDPPFNSLLFALLAAAGGLQGIYVLVMLVLLILAYRRRWRRLTVCGGIMFLACVLVLIVDAVLQLSPLLGAVTVVSMTLLLLAFVLWLSSPGGLGTLGAALLTLAAALALLASLILGTLNLTTMFLLMLLWTLVVLLICSSCSSCPLSKILLARLFLYALALLLLASALIAGGSILQTNFKSLSSTEFIPNLFCMLLLIVAGILFILAILTEWGSGNRTYGPVFMCLGGLLTMVAGAVWLTVMSNTLLSAWILTAGFLIFLIGFALFGVIRCCRYCCYYCLTLESEERPPTPYRNTV

SEQ ID NO: 28 - protein, 497 aa, Artificial Sequence
  LMP2 aa
MGSLEMVPMGAGPPSPGGDPDGYDGGNNSQYPSASGSSGNTPTPPNDEERESNEEPPPPYEDPYWGNGDRHSDYQPLGTQDQSLYLGLQHDGNDGLPPPPYSPRDDSSQHIYEEAGRGSMNPVCLPVIVAPYLFWLAAIAASCFTASVSTVVTATGLALSLLLLAAVASSYAAAQRKLLTPVTVLTAVVTFFAICLTWRIEDPPFNSLLFALLAAAGGLQGIYVLVMLVLLILAYRRRWRRLTVCGGIMFLACVLVLIVDAVLQLSPLLGAVTVVSMTLLLLAFVLWLSSPGGLGTLGAALLTLAAALALLASLILGTLNLTTMFLLMLLWTLVVLLICSSCSSCPLTKILLARLFLYALALLLLASALIAGGSILQTNFKSLSSTEFIPNLFCMLLLIVAGILFILAILTEWGSGNRTYGPVFMSLGGLLTMVAGAVWLTVMSNTLLSAWILTAGFLIFLIGFALFGVIRCCRYCCYYCLTLESEERPPTPYRNTV

SEQ ID NO: 29 - protein, 9 aa, Artificial Sequence
  antigen
FLYALALLL

SEQ ID NO: 30 - protein, 9 aa, Artificial Sequence
  antigen
PYLFWLAAI

SEQ ID NO: 31 - protein, 9 aa, Artificial Sequence
  antigen
TYGPVFMSL

SEQ ID NO: 32 - protein, 9 aa, Artificial Sequence
  antigen
TYGPVFMCL

SEQ ID NO: 33 - protein, 10 aa, Artificial Sequence
  antigen
SSCSSCPLSK

SEQ ID NO: 34 - protein, 10 aa, Artificial Sequence
  antigen
SSCSSCPLTK

SEQ ID NO: 35 - protein, 5 aa, Artificial Sequence
  CDR
TSINN

SEQ ID NO: 36 - protein, 6 aa, Artificial Sequence
  CDR
SSNFYA

SEQ ID NO: 37 - protein, 6 aa, Artificial Sequence
  CDR
DSASNY

SEQ ID NO: 38 - protein, 6 aa, Artificial Sequence
  CDR
NSAFQY

SEQ ID NO: 39 - protein, 5 aa, Artificial Sequence
  CDR
DSVNN

SEQ ID NO: 40 - protein, 5 aa, Artificial Sequence
  CDR
TTSDR

SEQ ID NO: 41 - protein, 7 aa, Artificial Sequence
  CDR
TRDTTYY

SEQ ID NO: 42 - protein, 6 aa, Artificial Sequence
  CDR
DSAIYN

SEQ ID NO: 43 - protein, 7 aa, Artificial Sequence
  CDR
TSDQSYG

SEQ ID NO: 44 - protein, 6 aa, Artificial Sequence
  CDR
NSASDY

SEQ ID NO: 45 - protein, 7 aa, Artificial Sequence
  CDR
IRSNERE

SEQ ID NO: 46 - protein, 7 aa, Artificial Sequence
  CDR
MTLNGDE

SEQ ID NO: 47 - protein, 7 aa, Artificial Sequence
  CDR
IRSNVGE

SEQ ID NO: 48 - protein, 6 aa, Artificial Sequence
  CDR
TYSSGN

SEQ ID NO: 49 - protein, 5 aa, Artificial Sequence
  CDR
IPSGT

SEQ ID NO: 50 - protein, 7 aa, Artificial Sequence
  CDR
LLSNGAV

SEQ ID NO: 51 - protein, 8 aa, Artificial Sequence
  CDR
RNSFDEQN

SEQ ID NO: 52 - protein, 7 aa, Artificial Sequence
  CDR
IQSSQRE

SEQ ID NO: 53 - protein, 8 aa, Artificial Sequence
  CDR
QGSYDEQN

SEQ ID NO: 54 - protein, 7 aa, Artificial Sequence
  CDR
IRSNMDK

SEQ ID NO: 55 - protein, 12 aa, Artificial Sequence
  CDR
ATEGDSGYSTLT

SEQ ID NO: 56 - protein, 12 aa, Artificial Sequence
  CDR
ATVGDSGYSTLT

SEQ ID NO: 57 - protein, 12 aa, Artificial Sequence
  CDR
ASTNSNSGYALN

SEQ ID NO: 58 - protein, 11 aa, Artificial Sequence
  CDR
AARGGGYSTLT

SEQ ID NO: 59 - protein, 11 aa, Artificial Sequence
  CDR
AMFRSTLGRLY

SEQ ID NO: 60 - protein, 9 aa, Artificial Sequence
  CDR
AVLNNNDMR

SEQ ID NO: 61 - protein, 9 aa, Artificial Sequence
  CDR
AVVDNNDMR

SEQ ID NO: 62 - protein, 11 aa, Artificial Sequence
  CDR
AVAMNRDDKII

SEQ ID NO: 63 - protein, 15 aa, Artificial Sequence
  CDR
AAREGFYQTGANNLF

SEQ ID NO: 64 - protein, 12 aa, Artificial Sequence
  CDR
AATAGGATNKLI

SEQ ID NO: 65 - protein, 10 aa, Artificial Sequence
  CDR
AVELTGNQFY

SEQ ID NO: 66 - protein, 10 aa, Artificial Sequence
  CDR
AVNTGFQKLV

SEQ ID NO: 67 - protein, 13 aa, Artificial Sequence
  CDR
ALSEPPSGTYKYI

SEQ ID NO: 68 - protein, 9 aa, Artificial Sequence
  CDR
AVLDNNDMR

SEQ ID NO: 69 - protein, 10 aa, Artificial Sequence
  CDR
AGKTSYDKVI

SEQ ID NO: 70 - protein, 14 aa, Artificial Sequence
  CDR
AMVSGAGGGADGLT

SEQ ID NO: 71 - protein, 11 aa, Artificial Sequence
  CDR
AETPGGYQKVT

SEQ ID NO: 72 - protein, 10 aa, Artificial Sequence
  CDR
AASNRDDKII

SEQ ID NO: 73 - protein, 13 aa, Artificial Sequence
  CDR
AVDIGTEYGNKLV

SEQ ID NO: 74 - protein, 5 aa, Artificial Sequence
  CDR
MNHEY

SEQ ID NO: 75 - protein, 6 aa, Artificial Sequence
  CDR
DFQATT

SEQ ID NO: 76 - protein, 5 aa, Artificial Sequence
  CDR
LNHDA

SEQ ID NO: 77 - protein, 5 aa, Artificial Sequence
  CDR
MGHRA

SEQ ID NO: 78 - protein, 5 aa, Artificial Sequence
  CDR
SGHKS

SEQ ID NO: 79 - protein, 5 aa, Artificial Sequence
  CDR
KGHSH

SEQ ID NO: 80 - protein, 5 aa, Artificial Sequence
  CDR
SGDLS

SEQ ID NO: 81 - protein, 5 aa, Artificial Sequence
  CDR
SNHLY

SEQ ID NO: 82 - protein, 5 aa, Artificial Sequence
  CDR
SGHVS

SEQ ID NO: 83 - protein, 5 aa, Artificial Sequence
  CDR
SGHAT

SEQ ID NO: 84 - protein, 5 aa, Artificial Sequence
  CDR
SGHNS

SEQ ID NO: 85 - protein, 6 aa, Artificial Sequence
  CDR
SVGAGI

SEQ ID NO: 86 - protein, 7 aa, Artificial Sequence
  CDR
SNEGSKA

SEQ ID NO: 87 - protein, 6 aa, Artificial Sequence
  CDR
SQIVND

SEQ ID NO: 88 - protein, 6 aa, Artificial Sequence
  CDR
SMNVEV

SEQ ID NO: 89 - protein, 6 aa, Artificial Sequence
  CDR
YSYEKL

SEQ ID NO: 90 - protein, 6 aa, Artificial Sequence
  CDR
YYEKEE

SEQ ID NO: 91 - protein, 6 aa, Artificial Sequence
  CDR
LQKENI

SEQ ID NO: 92 - protein, 6 aa, Artificial Sequence
  CDR
YYNGEE

SEQ ID NO: 93 - protein, 6 aa, Artificial Sequence
  CDR
FYNNEI

SEQ ID NO: 94 - protein, 6 aa, Artificial Sequence
  CDR
FQNEAQ

SEQ ID NO: 95 - protein, 6 aa, Artificial Sequence
  CDR
FQNNGV

SEQ ID NO: 96 - protein, 6 aa, Artificial Sequence
  CDR
FNNNVP

SEQ ID NO: 97 - protein, 12 aa, Artificial Sequence
  CDR
ASSYQGGSSGYT

SEQ ID NO: 98 - protein, 12 aa, Artificial Sequence
  CDR
ASSGQGGGYGYT

SEQ ID NO: 99 - protein, 15 aa, Artificial Sequence
  CDR
SARDTSGVNFYNEQF

SEQ ID NO: 100 - protein, 11 aa, Artificial Sequence
  CDR
ASAITGGTEAF

SEQ ID NO: 101 - protein, 16 aa, Artificial Sequence
  CDR
ASTPLPTSSGRLGEQY

SEQ ID NO: 102 - protein, 11 aa, Artificial Sequence
  CDR
ASSQGRWYEQY

SEQ ID NO: 103 - protein, 11 aa, Artificial Sequence
  CDR
ASSPGRWYEQF

SEQ ID NO: 104 - protein, 14 aa, Artificial Sequence
  CDR
ASSLDRDRNDYGYT

SEQ ID NO: 105 - protein, 14 aa, Artificial Sequence
  CDR
ASSPAPRAGNQPQH

SEQ ID NO: 106 - protein, 15 aa, Artificial Sequence
  CDR
ASSLYPPGHSNQPQH

SEQ ID NO: 107 - protein, 13 aa, Artificial Sequence
  CDR
ASSLEPGWGDTQY

SEQ ID NO: 108 - protein, 11 aa, Artificial Sequence
  CDR
ASSVGPWYEQY

SEQ ID NO: 109 - protein, 11 aa, Artificial Sequence
  CDR
ASSPGRFYEQY

SEQ ID NO: 110 - protein, 11 aa, Artificial Sequence
  CDR
ASSPGRWYEQY

SEQ ID NO: 111 - protein, 14 aa, Artificial Sequence
  CDR
ASSEGPTGTSYEQY

SEQ ID NO: 112 - protein, 13 aa, Artificial Sequence
  CDR
ASSQESGGTDTQY

SEQ ID NO: 113 - protein, 12 aa, Artificial Sequence
  CDR
ASSVFPTSVEQY

SEQ ID NO: 114 - protein, 14 aa, Artificial Sequence
  CDR
ASSIGVGLSNTEAF

SEQ ID NO: 115 - protein, 12 aa, Artificial Sequence
  CDR
ASSLWTSNSPLH

SEQ ID NO: 116 - protein, 13 aa, Artificial Sequence
  CDR
ASSLGAGHLWGYT

SEQ ID NO: 117 - protein, 12 aa, Artificial Sequence
  CDR
ASREGVGLYEQY

SEQ ID NO: 118 - DNA, 885 bp, Artificial Sequence
  A0201 NT
atgggcagccatagcatgcgttacttcttcaccagcgttagtcgccccggtcgcggtgaaccgcgctttatcgcagtgggttacgttgacgacacccagtttgtgcgttttgacagcgatgccgcaagccagcgtatggaaccgcgtgccccgtggattgaacaagaaggcccggaatactgggatggcgaaacccgcaaagttaaagcccacagccagacccatcgcgtggatctgggtactttacgtggctactataaccagagcgaagccggtagccataccgtgcagcgcatgtatggctgtgatgtgggcagtgattggcgctttctgcgcggctatcatcagtacgcctatgacggcaaggactacatcgctttaaaagaagatttacgtagttggaccgccgccgatatggcagcccagaccaccaaacataaatgggaagccgcccatgtggcagagcagctgcgcgcatatctggaaggcacatgcgtggaatggctgcgtcgctatctggagaacggcaaagaaactttacagcgcaccgacgcaccgaaaacccatatgacccaccatgccgtgagtgaccatgaagccactttacgctgttgggctttaagcttctatccggccgaaattactttaacttggcagcgcgatggtgaagaccagacccaagataccgagctggtggaaacccgtccggctggtgatggcacctttcagaaatgggtggccgttgtggtgccgagcggtcaagaacagcgctatacttgtcatgtgcagcatgagggcttaccgaaaccgctgactttacgctgggaaccgggatccggtttgaacgacatcttcgaagctcagaaaatcgaatggcacgaataa

SEQ ID NO: 119 - DNA, 885 bp, Artificial Sequence
  A2402 NT
atgggcagccacagtatgcgctacttcagcaccagcgttagtcgcccgggtcgtggtgaaccgcgttttatcgcagtgggctatgtggacgatacccagttcgttcgcttcgacagtgatgccgcaagtcagcgcatggaaccgcgtgccccgtggatcgaacaggaaggcccggaatactgggatgaggaaaccggcaaggtgaaagcacacagccagaccgaccgtgaaaacctgcgcattgccctgcgctattacaatcagagcgaagccggcagccacaccctgcagatgatgtttggttgcgatgtgggcagtgatggtcgctttctgcgcggctatcaccagtacgcctacgacggcaaggattatatcgccctgaaagaagacctgcgtagctggaccgcagccgatatggccgcccagattaccaaacgcaaatgggaggccgcacatgttgccgaacaacagcgcgcatatctggaaggtacctgtgtggatggtctgcgtcgctatctggaaaacggcaaagaaaccctgcagcgcaccgatcctccgaaaacccacatgacccaccacccgatcagcgaccatgaagccacactgcgttgctgggccctgggcttttacccggccgaaatcaccctgacctggcagcgcgatggcgaagatcagacccaggacaccgaactggtggaaacccgtccggcaggtgatggcacctttcagaaatgggtggcagtggttgtgccgagcggcgaagaacagcgttatacctgccatgtgcagcacgaaggtctgccgaaaccgctgaccctgcgctgggaacctggatccggtttgaacgacatcttcgaagctcagaaaatcgaatggcacgaataa

SEQ ID NO: 120 - DNA, 885 bp, Artificial Sequence
  A1101 NT
atgggtagccatagcatgcgctacttctataccagcgtgagtcgtccgggccgtggtgaacctcgctttattgccgtgggctatgtggatgacacccagttcgtgcgctttgatagcgatgccgcaagtcagcgcatggaaccgcgtgccccgtggattgaacaagaaggcccggaatattgggaccaagaaacacgcaacgttaaggcccagagccagacagatcgtgtggatctgggtacactgcgcggctattacaatcagagcgaggatggcagccacaccattcagatcatgtacggctgcgatgttggtccggacggtcgctttttacgtggctaccgtcaagatgcctatgatggcaaggactatatcgctttaaacgaggatctgcgcagttggaccgcagccgatatggccgcacagatcaccaaacgcaaatgggaagcagcacacgccgccgagcagcaacgtgcatatttagaaggtcgttgcgtggaatggctgcgccgctatctggagaatggcaaagaaactttacagcgtaccgatccgccgaaaacccatatgacccatcacccgatcagcgatcatgaggccactttacgttgttgggcactgggcttttatccggcagaaatcactttaacttggcagcgcgatggtgaagatcagacccaagataccgaactggtggaaacccgccccgctggtgatggcacctttcagaaatgggttgcagtggttgtgccgagcggcgaggaacagcgttacacttgtcacgttcagcatgaaggtttaccgaaaccgctgactttacgttgggaactgggatccggtttgaacgacatcttcgaagctcagaaaatcgaatggcacgaataa

SEQ ID NO: 121 - DNA, 306 bp, Artificial Sequence
  b2m NT
atggcaatccagcgtactccaaagattcaggtttactcacgtcatccagcagagaatggaaagtcaaatttcctgaattgctatgtgtctgggtttcatccatccgacattgaagttgacttactgaagaatggagagagaattgaaaaagtggagcattcagacttgtctttcagcaaggactggtctttctatctcttgtactacactgaattcacccccactgaaaaagatgagtatgcctgccgtgtgaaccatgtgactttgtcacagcccaagatagttaagtgggatcgagacatgtaa

SEQ ID NO: 122 - DNA, 1830 bp, Artificial Sequence
  E23 NT
atgagcatcggcctcctgtgctgtgcagccttgtctctcctgtgggcaggtccagtgaatgctggtgtcactcagaccccaaaattccaggtcctgaagacaggacagagcatgacactgcagtgtgcccaggatatgaaccatgaatacatgtcctggtatcgacaagacccaggcatggggctgaggctgattcattactcagttggtgctggtatcactgaccaaggagaagtccccaatggctacaatgtctccagatcaaccacagaggatttcccgctcaggctgctgtcggctgctccctcccagacatctgtgtacttctgtgccagcagttaccaagggggtagtagtggctacaccttcggttcggggaccaggttaaccgttgtagaggacctgaaaaacgtgttcccacccgaggtcgctgtgtttgagccatcagaagcagagatctcccacacccaaaaggccacactggtgtgcctggccacaggcttcttccccgaccacgtggagctgagctggtgggtgaatgggaaggaggtgcacagtggggtcagcacagacccgcagcccctcaaggagcagcccgccctcaatgactccagatactgcctgagcagccgcctgagggtctcggccaccttctggcagaacccccgcaaccacttccgctgtcaagtccagttctacgggctctcggagaatgacgagtggacccaggatagggccaaacccgtcacccagatcgtcagcgccgaggcctggggtagagcagactgtggctttacctcggtgtcctaccagcaaggggtcctgtctgccaccatcctctatgagatcctgctagggaaggccaccctgtatgctgtgctggtcagcgcccttgtgttgatggccatggtcaagagaaaggatttccggcggaaacggagcggaagcggagctactaacttcagcctgctgaagcaggctggagacgtggaggagaaccctggacctatggaaactctcctgggagtgtctttggtgattctatggcttcaactggctagggtgaacagtcaacagggagaagaggatcctcaggccttgagcatccaggagggtgaaaatgccaccatgaactgcagttacaaaactagtataaacaatttacagtggtatagacaaaattcaggtagaggccttgtccacctaattttaatacgttcaaatgaaagagagaaacacagtggaagattaagagtcacgcttgacacttccaagaaaagcagttccttgttgatcacggcttcccgggcagcagacactgcttcttacttctgtgctacggaaggggattcaggatacagcaccctcacctttgggaaggggactatgcttctagtctctccagatatccagaaccctgaccctgccgtgtaccagctgagagactctaaatccagtgacaagtctgtctgcctattcaccgattttgattctcaaacaaatgtgtcacaaagtaaggattctgatgtgtatatcacagacaaaactgtgctagacatgaggtctatggacttcaagagcaacagtgctgtggcctggagcaacaaatctgactttgcatgtgcaaacgccttcaacaacagcattattccagaagacaccttcttccccagcccagaaagttcctgtgatgtcaagctggtcgagaaaagctttgaaacagatacgaacctaaactttcaaaacctgtcagtgattgggttccgaatcctcctcctgaaagtggccgggtttaatctgctcatgacgctgcggctgtggtccagctga

SEQ ID NO: 123 - DNA, 1830 bp, Artificial Sequence
  E240 NT
atgagcatcggcctcctgtgctgtgcagccttgtctctcctgtgggcaggtccagtgaatgctggtgtcactcagaccccaaaattccaggtcctgaagacaggacagagcatgacactgcagtgtgcccaggatatgaaccatgaatacatgtcctggtatcgacaagacccaggcatggggctgaggctgattcattactcagttggtgctggtatcactgaccaaggagaagtccccaatggctacaatgtctccagatcaaccacagaggatttcccgctcaggctgctgtcggctgctccctcccagacatctgtgtacttctgtgccagcagcggacagggcggggggtatggctacaccttcggttcggggaccaggttaaccgttgtagaggacctgaaaaacgtgttcccacccgaggtcgctgtgtttgagccatcagaagcagagatctcccacacccaaaaggccacactggtgtgcctggccacaggcttcttccccgaccacgtggagctgagctggtgggtgaatgggaaggaggtgcacagtggggtcagcacagacccgcagcccctcaaggagcagcccgccctcaatgactccagatactgcctgagcagccgcctgagggtctcggccaccttctggcagaacccccgcaaccacttccgctgtcaagtccagttctacgggctctcggagaatgacgagtggacccaggatagggccaaacccgtcacccagatcgtcagcgccgaggcctggggtagagcagactgtggctttacctcggtgtcctaccagcaaggggtcctgtctgccaccatcctctatgagatcctgctagggaaggccaccctgtatgctgtgctggtcagcgcccttgtgttgatggccatggtcaagagaaaggatttccggcggaaacggagcggaagcggagctactaacttcagcctgctgaagcaggctggagacgtggaggagaaccctggacctatggaaactctcctgggagtgtctttggtgattctatggcttcaactggctagggtgaacagtcaacagggagaagaggatcctcaggccttgagcatccaggagggtgaaaatgccaccatgaactgcagttacaaaactagtataaacaatttacagtggtatagacaaaattcaggtagaggccttgtccacctaattttaatacgttcaaatgaaagagagaaacacagtggaagattaagagtcacgcttgacacttccaagaaaagcagttccttgttgatcacggcttcccgggcagcagacactgcttcttacttctgtgctacggtcggggattcaggatacagcaccctcacctttgggaaggggactatgcttctagtctctccagatatccagaaccctgaccctgccgtgtaccagctgagagactctaaatccagtgacaagtctgtctgcctattcaccgattttgattctcaaacaaatgtgtcacaaagtaaggattctgatgtgtatatcacagacaaaactgtgctagacatgaggtctatggacttcaagagcaacagtgctgtggcctggagcaacaaatctgactttgcatgtgcaaacgccttcaacaacagcattattccagaagacaccttcttccccagcccagaaagttcctgtgatgtcaagctggtcgagaaaagctttgaaacagatacgaacctaaactttcaaaacctgtcagtgattgggttccgaatcctcctcctgaaagtggccgggtttaatctgctcatgacgctgcggctgtggtccagctga

SEQ ID NO: 124 - DNA, 1842 bp, Artificial Sequence
  E29 NT
atgctgctgcttctgctgcttctggggccaggctccgggcttggtgctgtcgtctctcaacatccgagcagggttatctgtaagagtggaacctctgtgaagatcgagtgccgttccctggactttcaggccacaactatgttttggtatcgtcagttcccgaaaaagagtctcatgctgatggcaacttccaatgagggctccaaggccacatacgagcaaggcgtcgagaaggacaagtttctcatcaaccatgcaagcctgaccttgtccactctgacagtgaccagtgcccatcctgaagacagcagcttctacatctgcagtgctagagatactagcggggttaacttttacaatgagcagttcttcgggccagggacacggctcaccgtgctagaggacctgaaaaacgtgttcccacccgaggtcgctgtgtttgagccatcagaagcagagatctcccacacccaaaaggccacactggtgtgcctggccacaggcttcttccccgaccacgtggagctgagctggtgggtgaatgggaaggaggtgcacagtggggtcagcacagacccgcagcccctcaaggagcagcccgccctcaatgactccagatactgcctgagcagccgcctgagggtctcggccaccttctggcagaacccccgcaaccacttccgctgtcaagtccagttctacgggctctcggagaatgacgagtggacccaggatagggccaaacccgtcacccagatcgtcagcgccgaggcctggggtagagcagactgtggctttacctcggtgtcctaccagcaaggggtcctgtctgccaccatcctctatgagatcctgctagggaaggccaccctgtatgctgtgctggtcagcgcccttgtgttgatggccatggtcaagagaaaggatttccggcggaaacggagcggaagcggagctactaacttcagcctgctgaagcaggctggagacgtggaggagaaccctggacctatggagaagaatcctttggcagccccattactaatcctctggtttcatcttgactgcgtgagcagcatactgaacgtggaacaaagtcctcagtcactgcatgttcaggagggagacagcaccaatttcacctgcagcttcccttccagcaatttttatgccttacactggtacagatgggaaactgcaaaaagccccgaggccttgtttgtaatgactttaaatggggatgaaaagaagaaaggacgaataagtgccactcttaataccaaggagggttacagctatttgtacatcaaaggatcccagcctgaagactcagccacatacctctgtgcctccacgaactcaaattccgggtatgcactcaacttcggcaaaggcacctcgctgttggtcacaccccatatccagaaccctgaccctgccgtgtaccagctgagagactctaaatccagtgacaagtctgtctgcctattcaccgattttgattctcaaacaaatgtgtcacaaagtaaggattctgatgtgtatatcacagacaaaactgtgctagacatgaggtctatggacttcaagagcaacagtgctgtggcctggagcaacaaatctgactttgcatgtgcaaacgccttcaacaacagcattattccagaagacaccttcttccccagcccagaaagttcctgtgatgtcaagctggtcgagaaaagctttgaaacagatacgaacctaaactttcaaaacctgtcagtgattgggttccgaatcctcctcctgaaagtggccgggtttaatctgctcatgacgctgcggctgtggtccagctga

SEQ ID NO: 125 - DNA, 1824 bp, Artificial Sequence
  E180-1 NT
atgagcaaccaggtgctctgctgtgtggtcctttgtttcctgggagcaaacaccgtggatggtggaatcactcagtccccaaagtacctgttcagaaaggaaggacagaatgtgaccctgagttgtgaacagaatttgaaccacgatgccatgtactggtaccgacaggacccagggcaagggctgagattgatctactactcacagatagtaaatgactttcagaaaggagatatagctgaagggtacagcgtctctcgggagaagaaggaatcctttcctctcactgtgacatcggcccaaaagaacccgacagctttctatctctgtgccagtgcgattacggggggcactgaagctttctttggacaaggcaccagactcacagttgtagaggacctgaaaaacgtgttcccacccgaggtcgctgtgtttgagccatcagaagcagagatctcccacacccaaaaggccacactggtgtgcctggccacaggcttcttccccgaccacgtggagctgagctggtgggtgaatgggaaggaggtgcacagtggggtcagcacagacccgcagcccctcaaggagcagcccgccctcaatgactccagatactgcctgagcagccgcctgagggtctcggccaccttctggcagaacccccgcaaccacttccgctgtcaagtccagttctacgggctctcggagaatgacgagtggacccaggatagggccaaacccgtcacccagatcgtcagcgccgaggcctggggtagagcagactgtggctttacctcggtgtcctaccagcaaggggtcctgtctgccaccatcctctatgagatcctgctagggaaggccaccctgtatgctgtgctggtcagcgcccttgtgttgatggccatggtcaagagaaaggatttccggcggaaacggagcggaagcggagctactaacttcagcctgctgaagcaggctggagacgtggaggagaaccctggacctatgacatccattcgagctgtatttatattcctgtggctgcagctggacttggtgaatggagagaatgtggagcagcatccttcaaccctgagtgtccaggagggagacagcgctgttatcaagtgtacttattcagacagtgcctcaaactacttcccttggtataagcaagaacttggaaaaggacctcagcttattatagacattcgttcaaatgtgggcgaaaagaaagaccaacgaattgctgttacattgaacaagacagccaaacatttctccctgcacatcacagagacccaacctgaagactcggctgtctacttctgtgcagcccgcgggggaggatacagcaccctcacctttgggaaggggactatgcttctagtctctccagatatccagaaccctgaccctgccgtgtaccagctgagagactctaaatccagtgacaagtctgtctgcctattcaccgattttgattctcaaacaaatgtgtcacaaagtaaggattctgatgtgtatatcacagacaaaactgtgctagacatgaggtctatggacttcaagagcaacagtgctgtggcctggagcaacaaatctgactttgcatgtgcaaacgccttcaacaacagcattattccagaagacaccttcttccccagcccagaaagttcctgtgatgtcaagctggtcgagaaaagctttgaaacagatacgaacctaaactttcaaaacctgtcagtgattgggttccgaatcctcctcctgaaagtggccgggtttaatctgctcatgacgctgcggctgtggtccagctga

SEQ ID NO: 126 - DNA, 1845 bp, Artificial Sequence
  E44 NT
atgggcccccagctccttggctatgtggtcctttgccttctaggagcaggccccctggaagcccaagtgacccagaacccaagatacctcatcacagtgactggaaagaagttaacagtgacttgttctcagaatatgaaccatgagtatatgtcctggtatcgacaagacccagggctgggcttaaggcagatctactattcaatgaatgttgaggtgactgataagggagatgttcctgaagggtacaaagtctctcgaaaagagaagaggaatttccccctgatcctggagtcgcccagccccaaccagacctctctgtacttctgtgccagcactcccctacccacctctagcggaagacttggtgagcagtacttcgggccgggcaccaggctcacggtcacagaggacctgaaaaacgtgttcccacccgaggtcgctgtgtttgagccatcagaagcagagatctcccacacccaaaaggccacactggtgtgcctggccacaggcttcttccccgaccacgtggagctgagctggtgggtgaatgggaaggaggtgcacagtggggtcagcacagacccgcagcccctcaaggagcagcccgccctcaatgactccagatactgcctgagcagccgcctgagggtctcggccaccttctggcagaacccccgcaaccacttccgctgtcaagtccagttctacgggctctcggagaatgacgagtggacccaggatagggccaaacccgtcacccagatcgtcagcgccgaggcctggggtagagcagactgtggctttacctcggtgtcctaccagcaaggggtcctgtctgccaccatcctctatgagatcctgctagggaaggccaccctgtatgctgtgctggtcagcgcccttgtgttgatggccatggtcaagagaaaggatttccggcggaaacggagcggaagcggagctactaacttcagcctgctgaagcaggctggagacgtggaggagaaccctggacctatgatgaaatccttgagagttttactggtgatcctgtggcttcagttaagctgggtttggagccaacagaaggaggtggagcaggatcctggaccactcagtgttccagagggagccattgtttctctcaactgcacttacagcaacagtgcttttcaatacttcatgtggtacagacagtattccagaaaaggccctgagttgctgatgtacacatactccagtggtaacaaagaagatggaaggtttacagcacaggtcgataaatccagcaagtatatctccttgttcatcagagactcacagcccagtgattcagccacctacctctgtgcaatgttccgctcaaccctggggaggctatactttggaagaggaactcagttgactgtctggcctgatatccagaaccctgaccctgccgtgtaccagctgagagactctaaatccagtgacaagtctgtctgcctattcaccgattttgattctcaaacaaatgtgtcacaaagtaaggattctgatgtgtatatcacagacaaaactgtgctagacatgaggtctatggacttcaagagcaacagtgctgtggcctggagcaacaaatctgactttgcatgtgcaaacgccttcaacaacagcattattccagaagacaccttcttccccagcccagaaagttcctgtgatgtcaagctggtcgagaaaagctttgaaacagatacgaacctaaactttcaaaacctgtcagtgattgggttccgaatcctcctcctgaaagtggccgggtttaatctgctcatgacgctgcggctgtggtccagctga

SEQ ID NO: 127 - DNA, 1812 bp, Artificial Sequence
  E141 NT
atgggctgcaggctgctctgctgtgcggttctctgtctcctgggagcagttcccatagacactgaagttacccagacaccaaaacacctggtcatgggaatgacaaataagaagtctttgaaatgtgaacaacatatggggcacagggctatgtattggtacaagcagaaagctaagaagccaccggagctcatgtttgtctacagctatgagaaactctctataaatgaaagtgtgccaagtcgcttctcacctgaatgccccaacagctctctcttaaaccttcacctacacgccctgcagccagaagactcagccctgtatctctgcgccagcagccaggggcgatggtacgagcagtacttcgggccgggcaccaggctcacggtcacagaggacctgaaaaacgtgttcccacccgaggtcgctgtgtttgagccatcagaagcagagatctcccacacccaaaaggccacactggtgtgcctggccacaggcttcttccccgaccacgtggagctgagctggtgggtgaatgggaaggaggtgcacagtggggtcagcacagacccgcagcccctcaaggagcagcccgccctcaatgactccagatactgcctgagcagccgcctgagggtctcggccaccttctggcagaacccccgcaaccacttccgctgtcaagtccagttctacgggctctcggagaatgacgagtggacccaggatagggccaaacccgtcacccagatcgtcagcgccgaggcctggggtagagcagactgtggctttacctcggtgtcctaccagcaaggggtcctgtctgccaccatcctctatgagatcctgctagggaaggccaccctgtatgctgtgctggtcagcgcccttgtgttgatggccatggtcaagagaaaggatttccggcggaaacggagcggaagcggagctactaacttcagcctgctgaagcaggctggagacgtggaggagaaccctggacctatgaagaggatattgggagctctgctggggctcttgagtgcccaggtttgctgtgtgagaggaatacaagtggagcagagtcctccagacctgattctccaggagggagccaattccacgctgcggtgcaatttttctgactctgtgaacaatttgcagtggtttcatcaaaacccttggggacagctcatcaacctgttttacattccctcagggacaaaacagaatggaagattaagcgccacgactgtcgctacggaacgctacagcttattgtacatttcctcttcccagaccacagactcaggcgtttatttctgtgctgttctaaataacaatgacatgcgctttggagcagggaccagactgacagtaaaaccaaatatccagaaccctgaccctgccgtgtaccagctgagagactctaaatccagtgacaagtctgtctgcctattcaccgattttgattctcaaacaaatgtgtcacaaagtaaggattctgatgtgtatatcacagacaaaactgtgctagacatgaggtctatggacttcaagagcaacagtgctgtggcctggagcaacaaatctgactttgcatgtgcaaacgccttcaacaacagcattattccagaagacaccttcttccccagcccagaaagttcctgtgatgtcaagctggtcgagaaaagctttgaaacagatacgaacctaaactttcaaaacctgtcagtgattgggttccgaatcctcctcctgaaagtggccgggtttaatctgctcatgacgctgcggctgtggtccagctga

SEQ ID NO: 128 - DNA, 1812 bp, Artificial Sequence
  E149 NT
atgggctgcaggctgctctgctgtgcggttctctgtctcctgggagcagttcccatagacactgaagttacccagacaccaaaacacctggtcatgggaatgacaaataagaagtctttgaaatgtgaacaacatatggggcacagggctatgtattggtacaagcagaaagctaagaagccaccggagctcatgtttgtctacagctatgagaaactctctataaatgaaagtgtgccaagtcgcttctcacctgaatgccccaacagctctctcttaaaccttcacctacacgccctgcagccagaagactcagccctgtatctctgcgccagcagccccgggaggtggtatgagcagttcttcgggccagggacacggctcaccgtgctagaggacctgaaaaacgtgttcccacccgaggtcgctgtgtttgagccatcagaagcagagatctcccacacccaaaaggccacactggtgtgcctggccacaggcttcttccccgaccacgtggagctgagctggtgggtgaatgggaaggaggtgcacagtggggtcagcacagacccgcagcccctcaaggagcagcccgccctcaatgactccagatactgcctgagcagccgcctgagggtctcggccaccttctggcagaacccccgcaaccacttccgctgtcaagtccagttctacgggctctcggagaatgacgagtggacccaggatagggccaaacccgtcacccagatcgtcagcgccgaggcctggggtagagcagactgtggctttacctcggtgtcctaccagcaaggggtcctgtctgccaccatcctctatgagatcctgctagggaaggccaccctgtatgctgtgctggtcagcgcccttgtgttgatggccatggtcaagagaaaggatttccggcggaaacggagcggaagcggagctactaacttcagcctgctgaagcaggctggagacgtggaggagaaccctggacctatgaagaggatattgggagctctgctggggctcttgagtgcccaggtttgctgtgtgagaggaatacaagtggagcagagtcctccagacctgattctccaggagggagccaattccacgctgcggtgcaatttttctgactctgtgaacaatttgcagtggtttcatcaaaacccttggggacagctcatcaacctgttttacattccctcagggacaaaacagaatggaagattaagcgccacgactgtcgctacggaacgctacagcttattgtacatttcctcttcccagaccacagactcaggcgtttatttctgtgctgtggtcgataacaatgacatgcgctttggagcagggaccagactgacagtaaaaccaaatatccagaaccctgaccctgccgtgtaccagctgagagactctaaatccagtgacaagtctgtctgcctattcaccgattttgattctcaaacaaatgtgtcacaaagtaaggattctgatgtgtatatcacagacaaaactgtgctagacatgaggtctatggacttcaagagcaacagtgctgtggcctggagcaacaaatctgactttgcatgtgcaaacgccttcaacaacagcattattccagaagacaccttcttccccagcccagaaagttcctgtgatgtcaagctggtcgagaaaagctttgaaacagatacgaacctaaactttcaaaacctgtcagtgattgggttccgaatcctcctcctgaaagtggccgggtttaatctgctcatgacgctgcggctgtggtccagctga

SEQ ID NO: 129 - DNA, 1827 bp, Artificial Sequence
  E168 NT
atgggccctgggctcctctgctgggtgctgctttgtctcctgggagcaggcccagtggacgctggagtcacccaaagtcccacacacctgatcaaaacgagaggacagcacgtgactctgagatgctctcctatctctgggcacaagagtgtgtcctggtaccaacaggtcctgggtcaggggccccagtttatctttcagtattatgagaaagaagagagaggaagaggaaacttccctgatcgattctcagctcgccagttccctaactatagctctgagctgaatgtgaacgccttgttgctgggggactcggccctgtatctctgtgccagcagcttggatcgggacaggaatgactatggctacaccttcggttcggggaccaggttaaccgttgtagaggacctgaaaaacgtgttcccacccgaggtcgctgtgtttgagccatcagaagcagagatctcccacacccaaaaggccacactggtgtgcctggccacaggcttcttccccgaccacgtggagctgagctggtgggtgaatgggaaggaggtgcacagtggggtcagcacagacccgcagcccctcaaggagcagcccgccctcaatgactccagatactgcctgagcagccgcctgagggtctcggccaccttctggcagaacccccgcaaccacttccgctgtcaagtccagttctacgggctctcggagaatgacgagtggacccaggatagggccaaacccgtcacccagatcgtcagcgccgaggcctggggtagagcagactgtggctttacctcggtgtcctaccagcaaggggtcctgtctgccaccatcctctatgagatcctgctagggaaggccaccctgtatgctgtgctggtcagcgcccttgtgttgatggccatggtcaagagaaaggatttccggcggaaacggagcggaagcggagctactaacttcagcctgctgaagcaggctggagacgtggaggagaaccctggacctatgaagaagctactagcaatgattctgtggcttcaactagaccgattaagtggagagctgaaagtggaacaaaaccctctgttcctgagcatgcaggagggaaaaaactataccatctactgcaattattcaaccacttcagacagactgtattggtacaggcaggatcctgggaaaagtctggaatctctgtttgtgttgctatcaaatggagcagtgaagcaggagggacgattaatggcctcacttgataccaaagcccgtctcagcaccctccacatcacagctgccgtgcatgacctctctgccacctacttctgtgccgtagccatgaacagagatgacaagatcatctttggaaaagggacacgacttcatattctccccaatatccagaaccctgaccctgccgtgtaccagctgagagactctaaatccagtgacaagtctgtctgcctattcaccgattttgattctcaaacaaatgtgtcacaaagtaaggattctgatgtgtatatcacagacaaaactgtgctagacatgaggtctatggacttcaagagcaacagtgctgtggcctggagcaacaaatctgactttgcatgtgcaaacgccttcaacaacagcattattccagaagacaccttcttccccagcccagaaagttcctgtgatgtcaagctggtcgagaaaagctttgaaacagatacgaacctaaactttcaaaacctgtcagtgattgggttccgaatcctcctcctgaaagtggccgggtttaatctgctcatgacgctgcggctgtggtccagctga

SEQ ID NO: 130 - DNA, 1848 bp, Artificial Sequence
  E170 NT
atggacaccagagtactctgctgtgcggtcatctgtcttctgggggcaggtctctcaaatgccggcgtcatgcagaacccaagacacctggtcaggaggaggggacaggaggcaagactgagatgcagcccaatgaaaggacacagtcatgtttactggtatcggcagctcccagaggaaggtctgaaattcatggtttatctccagaaagaaaatatcatagatgagtcaggaatgccaaaggaacgattttctgctgaatttcccaaagagggccccagcatcctgaggatccagcaggtagtgcgaggagattcggcagcttatttctgtgccagctcacccgcccccagggcgggcaatcagccccagcattttggtgatgggactcgactctccatcctagaggacctgaaaaacgtgttcccacccgaggtcgctgtgtttgagccatcagaagcagagatctcccacacccaaaaggccacactggtgtgcctggccacaggcttcttccccgaccacgtggagctgagctggtgggtgaatgggaaggaggtgcacagtggggtcagcacagacccgcagcccctcaaggagcagcccgccctcaatgactccagatactgcctgagcagccgcctgagggtctcggccaccttctggcagaacccccgcaaccacttccgctgtcaagtccagttctacgggctctcggagaatgacgagtggacccaggatagggccaaacccgtcacccagatcgtcagcgccgaggcctggggtagagcagactgtggctttacctcggtgtcctaccagcaaggggtcctgtctgccaccatcctctatgagatcctgctagggaaggccaccctgtatgctgtgctggtcagcgcccttgtgttgatggccatggtcaagagaaaggatttccggcggaaacggagcggaagcggagctactaacttcagcctgctgaagcaggctggagacgtggaggagaaccctggacctatgacatccattcgagctgtatttatattcctgtggctgcagctggacttggtgaatggagagaatgtggagcagcatccttcaaccctgagtgtccaggagggagacagcgctgttatcaagtgtacttattcagacagtgcctcaaactacttcccttggtataagcaagaacttggaaaaagacctcagcttattatagacattcgttcaaatgtgggcgaaaagaaagaccaacgaattgctgttacattgaacaagacagccaaacatttctccctgcacatcacagagacccaacctgaagactcggctgtctacttctgtgcagcaagggagggtttttatcaaactggggcaaacaacctcttctttgggactggaacgagactcaccgttattccctatatccagaaccctgaccctgccgtgtaccagctgagagactctaaatccagtgacaagtctgtctgcctattcaccgattttgattctcaaacaaatgtgtcacaaagtaaggattctgatgtgtatatcacagacaaaactgtgctagacatgaggtctatggacttcaagagcaacagtgctgtggcctggagcaacaaatctgactttgcatgtgcaaacgccttcaacaacagcattattccagaagacaccttcttccccagcccagaaagttcctgtgatgtcaagctggtcgagaaaagctttgaaacagatacgaacctaaactttcaaaacctgtcagtgattgggttccgaatcctcctcctgaaagtggccgggtttaatctgctcatgacgctgcggctgtggtccagctga

SEQ ID NO: 131 - DNA, 1839 bp, Artificial Sequence
  E244/303 NT
atgggcccccagctccttggctatgtggtcctttgccttctaggagcaggccccctggaagcccaagtgacccagaacccaagatacctcatcacagtgactggaaagaagttaacagtgacttgttctcagaatatgaaccatgagtatatgtcctggtatcgacaagacccagggctgggcttaaggcagatctactattcaatgaatgttgaggtgactgataagggagatgttcctgaagggtacaaagtctctcgaaaagagaagaggaatttccccctgatcctggagtcgcccagccccaaccagacctctctgtacttctgtgccagcagtctatatccgcccggacactccaatcagccccagcattttggtgatgggactcgactctccatcctagaggacctgaaaaacgtgttcccacccgaggtcgctgtgtttgagccatcagaagcagagatctcccacacccaaaaggccacactggtgtgcctggccacaggcttcttccccgaccacgtggagctgagctggtgggtgaatgggaaggaggtgcacagtggggtcagcacagacccgcagcccctcaaggagcagcccgccctcaatgactccagatactgcctgagcagccgcctgagggtctcggccaccttctggcagaacccccgcaaccacttccgctgtcaagtccagttctacgggctctcggagaatgacgagtggacccaggatagggccaaacccgtcacccagatcgtcagcgccgaggcctggggtagagcagactgtggctttacctcggtgtcctaccagcaaggggtcctgtctgccaccatcctctatgagatcctgctagggaaggccaccctgtatgctgtgctggtcagcgcccttgtgttgatggccatggtcaagagaaaggatttccggcggaaacggagcggaagcggagctactaacttcagcctgctgaagcaggctggagacgtggaggagaaccctggacctatgacatccattcgagctgtatttatattcctgtggctgcagctggacttggtgaatggagagaatgtggagcagcatccttcaaccctgagtgtccaggagggagacagcgctgttatcaagtgtacttattcagacagtgcctcaaactacttcccttggtataagcaagaacttggaaaaagacctcagcttattatagacattcgttcaaatgtgggcgaaaagaaagaccaacgaattgctgttacattgaacaagacagccaaacatttctccctgcacatcacagagacccaacctgaagactcggctgtctacttctgtgcagcaaccgccggtggtgctacaaacaagctcatctttggaactggcactctgcttgctgtccagccaaatatccagaaccctgaccctgccgtgtaccagctgagagactctaaatccagtgacaagtctgtctgcctattcaccgattttgattctcaaacaaatgtgtcacaaagtaaggattctgatgtgtatatcacagacaaaactgtgctagacatgaggtctatggacttcaagagcaacagtgctgtggcctggagcaacaaatctgactttgcatgtgcaaacgccttcaacaacagcattattccagaagacaccttcttccccagcccagaaagttcctgtgatgtcaagctggtcgagaaaagctttgaaacagatacgaacctaaactttcaaaacctgtcagtgattgggttccgaatcctcctcctgaaagtggccgggtttaatctgctcatgacgctgcggctgtggtccagctga

SEQ ID NO: 132 - DNA, 1821 bp, Artificial Sequence
  E245 NT
atgggccctgggctcctctgctgggtgctgctttgtctcctgggagcaggcccagtggacgctggagtcacccaaagtcccacacacctgatcaaaacgagaggacagcacgtgactctgagatgctctcctatctctgggcacaagagtgtgtcctggtaccaacaggtcctgggtcaggggccccagtttatctttcagtattatgagaaagaagagagaggaagaggaaacttccctgatcgattctcagctcgccagttccctaactatagctctgagctgaatgtgaacgccttgttgctgggggactcggccctgtatctctgtgccagcagcttggagccgggatggggggatacgcagtattttggcccaggcacccggctgacagtgctcgaggacctgaaaaacgtgttcccacccgaggtcgctgtgtttgagccatcagaagcagagatctcccacacccaaaaggccacactggtgtgcctggccacaggcttcttccccgaccacgtggagctgagctggtgggtgaatgggaaggaggtgcacagtggggtcagcacagacccgcagcccctcaaggagcagcccgccctcaatgactccagatactgcctgagcagccgcctgagggtctcggccaccttctggcagaacccccgcaaccacttccgctgtcaagtccagttctacgggctctcggagaatgacgagtggacccaggatagggccaaacccgtcacccagatcgtcagcgccgaggcctggggtagagcagactgtggctttacctcggtgtcctaccagcaaggggtcctgtctgccaccatcctctatgagatcctgctagggaaggccaccctgtatgctgtgctggtcagcgcccttgtgttgatggccatggtcaagagaaaggatttccggcggaaacggagcggaagcggagctactaacttcagcctgctgaagcaggctggagacgtggaggagaaccctggacctatgaagaagctactagcaatgattctgtggcttcaactagaccggttaagtggagagctgaaagtggaacaaaaccctctgttcctgagcatgcaggagggaaaaaactataccatctactgcaattattcaaccacttcagacagactgtattggtacaggcaggatcctgggaaaagtctggaatctctgtttgtgttgctatcaaatggagcagtgaagcaggagggacgattaatggcctcacttgataccaaagcccgtctcagcaccctccacatcacagctgccgtgcatgacctctctgccacctacttctgtgccgtggaacttaccggtaaccagttctattttgggacagggacaagtttgacggtcattccaaatatccagaaccctgaccctgccgtgtaccagctgagagactctaaatccagtgacaagtctgtctgcctattcaccgattttgattctcaaacaaatgtgtcacaaagtaaggattctgatgtgtatatcacagacaaaactgtgctagacatgaggtctatggacttcaagagcaacagtgctgtggcctggagcaacaaatctgactttgcatgtgcaaacgccttcaacaacagcattattccagaagacaccttcttccccagcccagaaagttcctgtgatgtcaagctggtcgagaaaagctttgaaacagatacgaacctaaactttcaaaacctgtcagtgattgggttccgaatcctcctcctgaaagtggccgggtttaatctgctcatgacgctgcggctgtggtccagctga

SEQ ID NO: 133 - DNA, 1812 bp, Artificial Sequence
  E254 NT
atgggcttcaggctcctctgctgtgtggccttttgtctcctgggagcaggcccagtggattctggagtcacacaaaccccaaagcacctgatcacagcaactggacagcgagtgacgctgagatgctcccctaggtctggagacctctctgtgtactggtaccaacagagcctggaccagggcctccagttcctcattcagtattataatggagaagagagagcaaaaggaaacattcttgaacgattctccgcacaacagttccctgacttgcactctgaactaaacctgagctctctggagctgggggactcagctttgtatttctgtgccagcagcgtaggtccatggtacgagcagtacttcgggccgggcaccaggctcacggtcacagaggacctgaaaaacgtgttcccacccgaggtcgctgtgtttgagccatcagaagcagagatctcccacacccaaaaggccacactggtgtgcctggccacaggcttcttccccgaccacgtggagctgagctggtgggtgaatgggaaggaggtgcacagtggggtcagcacagacccgcagcccctcaaggagcagcccgccctcaatgactccagatactgcctgagcagccgcctgagggtctcggccaccttctggcagaacccccgcaaccacttccgctgtcaagtccagttctacgggctctcggagaatgacgagtggacccaggatagggccaaacccgtcacccagatcgtcagcgccgaggcctggggtagagcagactgtggctttacctcggtgtcctaccagcaaggggtcctgtctgccaccatcctctatgagatcctgctagggaaggccaccctgtatgctgtgctggtcagcgcccttgtgttgatggccatggtcaagagaaaggatttccggcggaaacggagcggaagcggagctactaacttcagcctgctgaagcaggctggagacgtggaggagaaccctggacctatgaagaggatattgggagctctgctggggctcttgagtgcccaggtttgctgtgtgagaggaatacaagtggagcagagtcctccagacctgattctccaggagggagccaattccacgctgcggtgcaatttttctgactctgtgaacaatttgcagtggtttcatcaaaacccttggggacagctcatcaacctgttttacattccctcagggacaaaacagaatggaagattaagcgccacgactgtcgctacggaacgctacagcttattgtacatttcctcttcccagaccacagactcaggcgtttatttctgtgctgtgctaaataacaatgacatgcgctttggagcagggaccagactgacagtaaaaccaaatatccagaaccctgaccctgccgtgtaccagctgagagactctaaatccagtgacaagtctgtctgcctattcaccgattttgattctcaaacaaatgtgtcacaaagtaaggattctgatgtgtatatcacagacaaaactgtgctagacatgaggtctatggacttcaagagcaacagtgctgtggcctggagcaacaaatctgactttgcatgtgcaaacgccttcaacaacagcattattccagaagacaccttcttccccagcccagaaagttcctgtgatgtcaagctggtcgagaaaagctttgaaacagatacgaacctaaactttcaaaacctgtcagtgattgggttccgaatcctcctcctgaaagtggccgggtttaatctgctcatgacgctgcggctgtggtccagctga

SEQ ID NO: 134 - DNA, 1812 bp, Artificial Sequence
  E301 NT
atgggctgcaggctgctctgctgtgcggttctctgtctcctgggagcagttcccatagacactgaagttacccagacaccaaaacacctggtcatgggaatgacaaataagaagtctttgaaatgtgaacaacatatggggcacagggctatgtattggtacaagcagaaagctaagaagccaccggagctcatgtttgtctacagctatgagaaactctctataaatgaaagtgtgccaagtcgcttctcacctgaatgccccaacagctctctcttaaaccttcacctacacgccctgcagccagaagactcagccctgtatctctgcgccagcagccccgggcgattctacgagcagtacttcgggccgggcaccaggctcacggtcacagaggacctgaaaaacgtgttcccacccgaggtcgctgtgtttgagccatcagaagcagagatctcccacacccaaaaggccacactggtgtgcctggccacaggcttcttccccgaccacgtggagctgagctggtgggtgaatgggaaggaggtgcacagtggggtcagcacagacccgcagcccctcaaggagcagcccgccctcaatgactccagatactgcctgagcagccgcctgagggtctcggccaccttctggcagaacccccgcaaccacttccgctgtcaagtccagttctacgggctctcggagaatgacgagtggacccaggatagggccaaacccgtcacccagatcgtcagcgccgaggcctggggtagagcagactgtggctttacctcggtgtcctaccagcaaggggtcctgtctgccaccatcctctatgagatcctgctagggaaggccaccctgtatgctgtgctggtcagcgcccttgtgttgatggccatggtcaagagaaaggatttccggcggaaacggagcggaagcggagctactaacttcagcctgctgaagcaggctggagacgtggaggagaaccctggacctatgaagaggatattgggagctctgctggggctcttgagtgcccaggtttgctgtgtgagaggaatacaagtggagcagagtcctccagacctgattctccaggagggagccaattccacgctgcggtgcaatttttctgactctgtgaacaatttgcagtggtttcatcaaaacccttggggacagctcatcaacctgttttacattccctcagggacaaaacagaatggaagattaagcgccacgactgtcgctacggaacgctacagcttattgtacatttcctcttcccagaccacagactcaggcgtttatttctgtgctgtccttaataacaatgacatgcgctttggagcagggaccagactgacagtaaaaccaaatatccagaaccctgaccctgccgtgtaccagctgagagactctaaatccagtgacaagtctgtctgcctattcaccgattttgattctcaaacaaatgtgtcacaaagtaaggattctgatgtgtatatcacagacaaaactgtgctagacatgaggtctatggacttcaagagcaacagtgctgtggcctggagcaacaaatctgactttgcatgtgcaaacgccttcaacaacagcattattccagaagacaccttcttccccagcccagaaagttcctgtgatgtcaagctggtcgagaaaagctttgaaacagatacgaacctaaactttcaaaacctgtcagtgattgggttccgaatcctcctcctgaaagtggccgggtttaatctgctcatgacgctgcggctgtggtccagctga

SEQ ID NO: 135 - DNA, 1812 bp, Artificial Sequence
  E304 NT
atgggctgcaggctgctctgctgtgcggttctctgtctcctgggagcagttcccatagacactgaagttacccagacaccaaaacacctggtcatgggaatgacaaataagaagtctttgaaatgtgaacaacatatggggcacagggctatgtattggtacaagcagaaagctaagaagccaccggagctcatgtttgtctacagctatgagaaactctctataaatgaaagtgtgccaagtcgcttctcacctgaatgccccaacagctctctcttaaaccttcacctacacgccctgcagccagaagactcagccctgtatctctgcgccagcagcccggggcggtggtacgagcagtacttcgggccgggcaccaggctcacggtcacagaggacctgaaaaacgtgttcccacccgaggtcgctgtgtttgagccatcagaagcagagatctcccacacccaaaaggccacactggtgtgcctggccacaggcttcttccccgaccacgtggagctgagctggtgggtgaatgggaaggaggtgcacagtggggtcagcacagacccgcagcccctcaaggagcagcccgccctcaatgactccagatactgcctgagcagccgcctgagggtctcggccaccttctggcagaacccccgcaaccacttccgctgtcaagtccagttctacgggctctcggagaatgacgagtggacccaggatagggccaaacccgtcacccagatcgtcagcgccgaggcctggggtagagcagactgtggctttacctcggtgtcctaccagcaaggggtcctgtctgccaccatcctctatgagatcctgctagggaaggccaccctgtatgctgtgctggtcagcgcccttgtgttgatggccatggtcaagagaaaggatttccggcggaaacggagcggaagcggagctactaacttcagcctgctgaagcaggctggagacgtggaggagaaccctggacctatgaagaggatattgggagctctgctggggctcttgagtgcccaggtttgctgtgtgagaggaatacaagtggagcagagtcctccagacctgattctccaggagggagccaattccacgctgcggtgcaatttttctgactctgtgaacaatttgcagtggtttcatcaaaacccttggggacagctcatcaacctgttttacattccctcagggacaaaacagaatggaagattaagcgccacgactgtcgctacggaacgctacagcttattgtacatttcctcttcccagaccacagactcaggcgtttatttctgtgctgtggtcgataacaatgacatgcgctttggagcagggaccagactgacagtaaaaccaaatatccagaaccctgaccctgccgtgtaccagctgagagactctaaatccagtgacaagtctgtctgcctattcaccgattttgattctcaaacaaatgtgtcacaaagtaaggattctgatgtgtatatcacagacaaaactgtgctagacatgaggtctatggacttcaagagcaacagtgctgtggcctggagcaacaaatctgactttgcatgtgcaaacgccttcaacaacagcattattccagaagacaccttcttccccagcccagaaagttcctgtgatgtcaagctggtcgagaaaagctttgaaacagatacgaacctaaactttcaaaacctgtcagtgattgggttccgaatcctcctcctgaaagtggccgggtttaatctgctcatgacgctgcggctgtggtccagctga

SEQ ID NO: 136 - DNA, 1827 bp, Artificial Sequence
  E305 NT
atggatacctggctcgtatgctgggcaatttttagtctcttgaaagcaggactcacagaacctgaagtcacccagactcccagccatcaggtcacacagatgggacaggaagtgatcttgcgctgtgtccccatctctaatcacttatacttctattggtacagacaaatcttggggcagaaagtcgagtttctggtttccttttataataatgaaatctcagagaagtctgaaatattcgatgatcaattctcagttgaaaggcctgatggatcaaatttcactctgaagatccggtccacaaagctggaggactcagccatgtacttctgtgccagcagtgaaggtccgacaggtacttcctacgagcagtacttcgggccgggcaccaggctcacggtcacagaggacctgaaaaacgtgttcccacccgaggtcgctgtgtttgagccatcagaagcagagatctcccacacccaaaaggccacactggtgtgcctggccacaggcttcttccccgaccacgtggagctgagctggtgggtgaatgggaaggaggtgcacagtggggtcagcacagacccgcagcccctcaaggagcagcccgccctcaatgactccagatactgcctgagcagccgcctgagggtctcggccaccttctggcagaacccccgcaaccacttccgctgtcaagtccagttctacgggctctcggagaatgacgagtggacccaggatagggccaaacccgtcacccagatcgtcagcgccgaggcctggggtagagcagactgtggctttacctcggtgtcctaccagcaaggggtcctgtctgccaccatcctctatgagatcctgctagggaaggccaccctgtatgctgtgctggtcagcgcccttgtgttgatggccatggtcaagagaaaggatttccggcggaaacggagcggaagcggagctactaacttcagcctgctgaagcaggctggagacgtggaggagaaccctggacctatgaagaagctactagcaatgattctgtggcttcaactagaccggttaagtggagagctgaaagtggaacaaaaccctctgttcctgagcatgcaggagggaaaaaactataccatctactgcaattattcaaccacttcagacagactgtattggtacaggcaggatcctgggaaaagtctggaatctctgtttgtgttgctatcaaatggagcagtgaagcaggagggacgattaatggcctcacttgataccaaagcccgtctcagcaccctccacatcacagctgccgtgcatgacctctctgccacctacttctgtgccgtgaacacaggctttcagaaacttgtatttggaactggcacccgacttctggtcagtccaaatatccagaaccctgaccctgccgtgtaccagctgagagactctaaatccagtgacaagtctgtctgcctattcaccgattttgattctcaaacaaatgtgtcacaaagtaaggattctgatgtgtatatcacagacaaaactgtgctagacatgaggtctatggacttcaagagcaacagtgctgtggcctggagcaacaaatctgactttgcatgtgcaaacgccttcaacaacagcattattccagaagacaccttcttccccagcccagaaagttcctgtgatgtcaagctggtcgagaaaagctttgaaacagatacgaacctaaactttcaaaacctgtcagtgattgggttccgaatcctcctcctgaaagtggccgggtttaatctgctcatgacgctgcggctgtggtccagctga

SEQ ID NO: 137 - DNA, 1848 bp, Artificial Sequence
  E307 NT
atgggcaccaggctcctctgctgggtggtcctgggtttcctagggacagatcacacaggtgctggagtctcccagtcccctaggtacaaagtcgcaaagagaggacaggatgtagctctcaggtgtgatccaatttcgggtcatgtatcccttttttggtaccaacaggccctggggcaggggccagagtttctgacttatttccagaatgaagctcaactagacaaatcggggctgcccagtgatcgcttctttgcagaaaggcctgagggatccgtctccactctgaagatccagcgcacacagcaggaggactccgccgtgtatctctgtgccagcagccaggagagcggggggacagatacgcagtattttggcccaggcacccggctgacagtgctcgaggacctgaaaaacgtgttcccacccgaggtcgctgtgtttgagccatcagaagcagagatctcccacacccaaaaggccacactggtgtgcctggccacaggcttcttccccgaccacgtggagctgagctggtgggtgaatgggaaggaggtgcacagtggggtcagcacagacccgcagcccctcaaggagcagcccgccctcaatgactccagatactgcctgagcagccgcctgagggtctcggccaccttctggcagaacccccgcaaccacttccgctgtcaagtccagttctacgggctctcggagaatgacgagtggacccaggatagggccaaacccgtcacccagatcgtcagcgccgaggcctggggtagagcagactgtggctttacctcggtgtcctaccagcaaggggtcctgtctgccaccatcctctatgagatcctgctagggaaggccaccctgtatgctgtgctggtcagcgcccttgtgttgatggccatggtcaagagaaaggatttccggcggaaacggagcggaagcggagctactaacttcagcctgctgaagcaggctggagacgtggaggagaaccctggacctatgctgactgccagcctgttgagggcagtcatagcctccatctgtgttgtatccagcatggctcagaaggtaactcaagcgcagactgaaatttctgtggtggagaaggaggatgtgaccttggactgtgtgtatgaaacccgtgatactacttattacttattctggtacaagcaaccaccaagtggagaattggttttccttattcgtcggaactcttttgatgagcaaaatgaaataagtggtcggtattcttggaacttccagaaatccaccagttccttcaacttcaccatcacagcctcacaagtcgtggactcagcagtatacttctgtgctctgagtgagccgccctcaggaacctacaaatacatctttggaacaggcaccaggctgaaggttttagcaaatatccagaaccctgaccctgccgtgtaccagctgagagactctaaatccagtgacaagtctgtctgcctattcaccgattttgattctcaaacaaatgtgtcacaaagtaaggattctgatgtgtatatcacagacaaaactgtgctagacatgaggtctatggacttcaagagcaacagtgctgtggcctggagcaacaaatctgactttgcatgtgcaaacgccttcaacaacagcattattccagaagacaccttcttccccagcccagaaagttcctgtgatgtcaagctggtcgagaaaagctttgaaacagatacgaacctaaactttcaaaacctgtcagtgattgggttccgaatcctcctcctgaaagtggccgggtttaatctgctcatgacgctgcggctgtggtccagctga

SEQ ID NO: 138 - DNA, 1812 bp, Artificial Sequence
  E314 NT
atgggctgcaggctgctctgctgtgcggttctctgtctcctgggagcagttcccatagacactgaagttacccagacaccaaaacacctggtcatgggaatgacaaataagaagtctttgaaatgtgaacaacatatggggcacagggctatgtattggtacaagcagaaagctaagaagccaccggagctcatgtttgtctacagctatgagaaactctctataaatgaaagtgtgccaagtcgcttctcacctgaatgccccaacagctctctcttaaaccttcacctacacgccctgcagccagaagactcagccctgtatctctgcgccagcagccaagggcggtggtacgagcagtacttcgggccgggcaccaggctcacggtcacagaggacctgaaaaacgtgttcccacccgaggtcgctgtgtttgagccatcagaagcagagatctcccacacccaaaaggccacactggtgtgcctggccacaggcttcttccccgaccacgtggagctgagctggtgggtgaatgggaaggaggtgcacagtggggtcagcacagacccgcagcccctcaaggagcagcccgccctcaatgactccagatactgcctgagcagccgcctgagggtctcggccaccttctggcagaacccccgcaaccacttccgctgtcaagtccagttctacgggctctcggagaatgacgagtggacccaggatagggccaaacccgtcacccagatcgtcagcgccgaggcctggggtagagcagactgtggctttacctcggtgtcctaccagcaaggggtcctgtctgccaccatcctctatgagatcctgctagggaaggccaccctgtatgctgtgctggtcagcgcccttgtgttgatggccatggtcaagagaaaggatttccggcggaaacggagcggaagcggagctactaacttcagcctgctgaagcaggctggagacgtggaggagaaccctggacctatgaagaggatattgggagctctgctggggctcttgagtgcccaggtttgctgtgtgagaggaatacaagtggagcagagtcctccagacctgattctccaggagggagccaattccacgctgcggtgcaatttttctgactctgtgaacaatttgcagtggtttcatcaaaacccttggggacagctcatcaacctgttttacattccctcagggacaaaacagaatggaagattaagcgccacgactgtcgctacggaacgctacagcttattgtacatttcctcttcccagaccacagactcaggcgtttatttctgtgctgtgctagataacaatgacatgcgctttggagcagggaccagactgacagtaaaaccaaatatccagaaccctgaccctgccgtgtaccagctgagagactctaaatccagtgacaagtctgtctgcctattcaccgattttgattctcaaacaaatgtgtcacaaagtaaggattctgatgtgtatatcacagacaaaactgtgctagacatgaggtctatggacttcaagagcaacagtgctgtggcctggagcaacaaatctgactttgcatgtgcaaacgccttcaacaacagcattattccagaagacaccttcttccccagcccagaaagttcctgtgatgtcaagctggtcgagaaaagctttgaaacagatacgaacctaaactttcaaaacctgtcagtgattgggttccgaatcctcctcctgaaagtggccgggtttaatctgctcatgacgctgcggctgtggtccagctga

SEQ ID NO: 139 - DNA, 1827 bp, Artificial Sequence
  E315 NT
atgggcaccaggctcctctgctgggcggccctctgtctcctgggagcagaactcacagaagctggagttgcccagtctcccagatataagattatagagaaaaggcagagtgtggctttttggtgcaatcctatatctggccatgctaccctttactggtaccagcagatcctgggacagggcccaaagcttctgattcagtttcagaataacggtgtagtggatgattcacagttgcctaaggatcgattttctgcagagaggctcaaaggagtagactccactctcaagatccagcctgcaaagcttgaggactcggccgtgtatctctgtgccagcagcgtcttccctactagcgtcgagcagtacttcgggccgggcaccaggctcacggtcacagaggacctgaaaaacgtgttcccacccgaggtcgctgtgtttgagccatcagaagcagagatctcccacacccaaaaggccacactggtgtgcctggccacaggcttcttccccgaccacgtggagctgagctggtgggtgaatgggaaggaggtgcacagtggggtcagcacagacccgcagcccctcaaggagcagcccgccctcaatgactccagatactgcctgagcagccgcctgagggtctcggccaccttctggcagaacccccgcaaccacttccgctgtcaagtccagttctacgggctctcggagaatgacgagtggacccaggatagggccaaacccgtcacccagatcgtcagcgccgaggcctggggtagagcagactgtggctttacctcggtgtcctaccagcaaggggtcctgtctgccaccatcctctatgagatcctgctagggaaggccaccctgtatgctgtgctggtcagcgcccttgtgttgatggccatggtcaagagaaaggatttccggcggaaacggagcggaagcggagctactaacttcagcctgctgaagcaggctggagacgtggaggagaaccctggacctatggagaccctcttgggcctgcttatcctttggctgcagctgcaatgggtgagcagcaaacaggaggtgacgcagattcctgcagctctgagtgtcccagaaggagaaaacttggttctcaactgcagtttcactgatagcgctatttacaacctccagtggtttaggcaggaccctgggaaaggtctcacatctctgttgcttattcagtcaagtcagagagagcaaacaagtggaagacttaatgcctcgctggataaatcatcaggacgtagtactttatacattgcagcttctcagcctggtgactcagccacctacctctgtgctggtaaaacctcctacgacaaggtgatatttgggccagggacaagcttatcagtcattccaaatatccagaaccctgaccctgccgtgtaccagctgagagactctaaatccagtgacaagtctgtctgcctattcaccgattttgattctcaaacaaatgtgtcacaaagtaaggattctgatgtgtatatcacagacaaaactgtgctagacatgaggtctatggacttcaagagcaacagtgctgtggcctggagcaacaaatctgactttgcatgtgcaaacgccttcaacaacagcattattccagaagacaccttcttccccagcccagaaagttcctgtgatgtcaagctggtcgagaaaagctttgaaacagatacgaacctaaactttcaaaacctgtcagtgattgggttccgaatcctcctcctgaaagtggccgggtttaatctgctcatgacgctgcggctgtggtccagctga

SEQ ID NO: 140 - DNA, 1851 bp, Artificial Sequence
  E316 NT
atgagcaaccaggtgctctgctgtgtggtcctttgtctcctgggagcaaacaccgtggatggtggaatcactcagtccccgaagtacctgttcagaaaggaaggacagaatgtgaccctgagttgtgaacagaatttgaaccacgatgccatgtactggtaccgacaggacccagggcaagggctgagattgatctactactcacagatagtaaatgactttcagaaaggagatatagctgaagggtacagcgtctctcgggagaagaaggaatcctttcctctcactgtgacatcggcccaaaagaacccgacagctttctatctctgtgccagtagtatcggtgtggggttatctaacactgaagctttctttggacaaggcaccagactcacagttgtagaggacctgaaaaacgtgttcccacccgaggtcgctgtgtttgagccatcagaagcagagatctcccacacccaaaaggccacactggtgtgcctggccacaggcttcttccccgaccacgtggagctgagctggtgggtgaatgggaaggaggtgcacagtggggtcagcacagacccgcagcccctcaaggagcagcccgccctcaatgactccagatactgcctgagcagccgcctgagggtctcggccaccttctggcagaacccccgcaaccacttccgctgtcaagtccagttctacgggctctcggagaatgacgagtggacccaggatagggccaaacccgtcacccagatcgtcagcgccgaggcctggggtagagcagactgtggctttacctcggtgtcctaccagcaaggggtcctgtctgccaccatcctctatgagatcctgctagggaaggccaccctgtatgctgtgctggtcagcgcccttgtgttgatggccatggtcaagagaaaggatttccggcggaaacggagcggaagcggagctactaacttcagcctgctgaagcaggctggagacgtggaggagaaccctggacctatgtcactttctagcctgctgaaggtggtcacagcttcactgtggctaggacctggcattgcccagaagataactcaaacccaaccaggaatgttcgtgcaggaaaaggaggctgtgactctggactgcacatatgacaccagtgatcaaagttatggtctattctggtacaagcagcccagcagtggggaaatgatttttcttatttatcaggggtcttatgacgagcaaaatgcaacagaaggtcgctactcattgaatttccagaaggcaagaaaatccgccaaccttgtcatctccgcttcacaactgggggactcagcaatgtatttctgtgcaatggtctcgggggcaggaggaggtgctgacggactcacctttggcaaagggactcatctaatcatccagccctatatccagaaccctgaccctgccgtgtaccagctgagagactctaaatccagtgacaagtctgtctgcctattcaccgattttgattctcaaacaaatgtgtcacaaagtaaggattctgatgtgtatatcacagacaaaactgtgctagacatgaggtctatggacttcaagagcaacagtgctgtggcctggagcaacaaatctgactttgcatgtgcaaacgccttcaacaacagcattattccagaagacaccttcttccccagcccagaaagttcctgtgatgtcaagctggtcgagaaaagctttgaaacagatacgaacctaaactttcaaaacctgtcagtgattgggttccgaatcctcctcctgaaagtggccgggtttaatctgctcatgacgctgcggctgtggtccagctga

SEQ ID NO: 141 - DNA, 1830 bp, Artificial Sequence
  E317 NT
atgggcccccagctccttggctatgtggtcctttgccttctaggagcaggccccctggaagcccaagtgacccagaacccaagatacctcatcacagtgactggaaagaagttaacagtgacttgttctcagaatatgaaccatgagtatatgtcctggtatcgacaagacccagggctgggcttaaggcagatctactattcaatgaatgttgaggtgactgataagggagatgttcctgaagggtacaaagtctctcgaaaagagaagaggaatttccccctgatcctggagtcgcccagccccaaccagacctctctgtacttctgtgccagcagtttatggacaagtaattcacccctccactttgggaacgggaccaggctcactgtgacagaggacctgaaaaacgtgttcccacccgaggtcgctgtgtttgagccatcagaagcagagatctcccacacccaaaaggccacactggtgtgcctggccacaggcttcttccccgaccacgtggagctgagctggtgggtgaatgggaaggaggtgcacagtggggtcagcacagacccgcagcccctcaaggagcagcccgccctcaatgactccagatactgcctgagcagccgcctgagggtctcggccaccttctggcagaacccccgcaaccacttccgctgtcaagtccagttctacgggctctcggagaatgacgagtggacccaggatagggccaaacccgtcacccagatcgtcagcgccgaggcctggggtagagcagactgtggctttacctcggtgtcctaccagcaaggggtcctgtctgccaccatcctctatgagatcctgctagggaaggccaccctgtatgctgtgctggtcagcgcccttgtgttgatggccatggtcaagagaaaggatttccggcggaaacggagcggaagcggagctactaacttcagcctgctgaagcaggctggagacgtggaggagaaccctggacctatggcaggcattcgagctttatttatgtacttgtggctgcagctggactgggtgagcagaggagagagtgtggggctgcatcttcctaccctgagtgtccaggagggtgacaactctattatcaactgtgcttattcaaacagcgcctcagactacttcatttggtacaagcaagaatctggaaaaggtcctcaattcattatagacattcgttcaaatatggacaaaaggcaaggccaaagagtcaccgttttattgaataagacagtgaaacatctctctctgcaaattgcagctactcaacctggagactcagctgtctacttttgtgcagagaccccagggggttaccagaaagttacctttggaactggaacaaagctccaagtcatcccaaatatccagaaccctgaccctgccgtgtaccagctgagagactctaaatccagtgacaagtctgtctgcctattcaccgattttgattctcaaacaaatgtgtcacaaagtaaggattctgatgtgtatatcacagacaaaactgtgctagacatgaggtctatggacttcaagagcaacagtgctgtggcctggagcaacaaatctgactttgcatgtgcaaacgccttcaacaacagcattattccagaagacaccttcttccccagcccagaaagttcctgtgatgtcaagctggtcgagaaaagctttgaaacagatacgaacctaaactttcaaaacctgtcagtgattgggttccgaatcctcctcctgaaagtggccgggtttaatctgctcatgacgctgcggctgtggtccagctga

SEQ ID NO: 142 - DNA, 1830 bp, Artificial Sequence
  E318 NT
atggactcctggaccttctgctgtgtgtccctttgcatcctggtagcgaagcatacagatgctggagttatccagtcaccccgccatgaggtgacagagatgggacaagaagtgactctgagatgtaaaccaatttcaggccacaactcccttttctggtacagacagaccatgatgcggggactggagttgctcatttactttaacaacaacgttccgatagatgattcagggatgcccgaggatcgattctcagctaagatgcctaatgcatcattctccactctgaagatccagccctcagaacccagggactcagctgtgtacttctgtgccagcagtttgggggcagggcatttatggggctacaccttcggttcggggaccaggttaaccgttgtagaggacctgaaaaacgtgttcccacccgaggtcgctgtgtttgagccatcagaagcagagatctcccacacccaaaaggccacactggtgtgcctggccacaggcttcttccccgaccacgtggagctgagctggtgggtgaatgggaaggaggtgcacagtggggtcagcacagacccgcagcccctcaaggagcagcccgccctcaatgactccagatactgcctgagcagccgcctgagggtctcggccaccttctggcagaacccccgcaaccacttccgctgtcaagtccagttctacgggctctcggagaatgacgagtggacccaggatagggccaaacccgtcacccagatcgtcagcgccgaggcctggggtagagcagactgtggctttacctcggtgtcctaccagcaaggggtcctgtctgccaccatcctctatgagatcctgctagggaaggccaccctgtatgctgtgctggtcagcgcccttgtgttgatggccatggtcaagagaaaggatttccggcggaaacggagcggaagcggagctactaacttcagcctgctgaagcaggctggagacgtggaggagaaccctggacctatgacatccattcgagctgtatttatattcctgtggctgcagctggacttggtgaatggagagaatgtggagcagcatccttcaaccctgagtgtccaggagggagacagcgctgttatcaagtgtacttattcagacagtgcctcaaactacttcccttggtataagcaagaacttggaaaaagacctcagcttattatagacattcgttcaaatgtgggcgaaaagaaagaccaacgaattgctgttacattgaacaagacagccaaacatttctccctgcacatcacagagacccaacctgaagactcggctgtctacttctgtgcagcttcgaacagagatgacaagatcatctttggaaaagggacacgacttcatattctccccaatatccagaaccctgaccctgccgtgtaccagctgagagactctaaatccagtgacaagtctgtctgcctattcaccgattttgattctcaaacaaatgtgtcacaaagtaaggattctgatgtgtatatcacagacaaaactgtgctagacatgaggtctatggacttcaagagcaacagtgctgtggcctggagcaacaaatctgactttgcatgtgcaaacgccttcaacaacagcattattccagaagacaccttcttccccagcccagaaagttcctgtgatgtcaagctggtcgagaaaagctttgaaacagatacgaacctaaactttcaaaacctgtcagtgattgggttccgaatcctcctcctgaaagtggccgggtttaatctgctcatgacgctgcggctgtggtccagctga

SEQ ID NO: 143 - DNA, 1830 bp, Artificial Sequence
  E320 NT
atgggcaccaggctcctctgctgggtggtcctgggtttcctagggacagatcacacaggtgctggagtctcccagtcccctaggtacaaagtcgcaaagagaggacaggatgtagctctcaggtgtgatccaatttcgggtcatgtatcccttttttggtaccaacaggccctggggcaggggccagagtttctgacttatttccagaatgaagctcaactagacaaatcggggctgcccagtgatcgcttctttgcagaaaggcctgagggatccgtctccactctgaagatccagcgcacacagcaggaggactccgccgtgtatctctgtgccagcagggaaggggtggggctctacgagcagtacttcgggccgggcaccaggctcacggtcacagaggacctgaaaaacgtgttcccacccgaggtcgctgtgtttgagccatcagaagcagagatctcccacacccaaaaggccacactggtgtgcctggccacaggcttcttccccgaccacgtggagctgagctggtgggtgaatgggaaggaggtgcacagtggggtcagcacagacccgcagcccctcaaggagcagcccgccctcaatgactccagatactgcctgagcagccgcctgagggtctcggccaccttctggcagaacccccgcaaccacttccgctgtcaagtccagttctacgggctctcggagaatgacgagtggacccaggatagggccaaacccgtcacccagatcgtcagcgccgaggcctggggtagagcagactgtggctttacctcggtgtcctaccagcaaggggtcctgtctgccaccatcctctatgagatcctgctagggaaggccaccctgtatgctgtgctggtcagcgcccttgtgttgatggccatggtcaagagaaaggatttccggcggaaacggagcggaagcggagctactaacttcagcctgctgaagcaggctggagacgtggaggagaaccctggacctatgaagaagctactagcaatgattctgtggcttcaactagaccggttaagtggagagctgaaagtggaacaaaaccctctgttcctgagcatgcaggagggaaaaaactataccatctactgcaattattcaaccacttcagacagactgtattggtacaggcaggatcctgggaaaagtctggaatctctgtttgtgttgctatcaaatggagcagtgaagcaggagggacgattaatggcctcacttgataccaaagcccgtctcagcaccctccacatcacagctgccgtgcatgacctctctgccacctacttctgtgccgtggacataggtacggaatatggaaacaagctggtctttggcgcaggaaccattctgagagtcaagtcctatatccagaaccctgaccctgccgtgtaccagctgagagactctaaatccagtgacaagtctgtctgcctattcaccgattttgattctcaaacaaatgtgtcacaaagtaaggattctgatgtgtatatcacagacaaaactgtgctagacatgaggtctatggacttcaagagcaacagtgctgtggcctggagcaacaaatctgactttgcatgtgcaaacgccttcaacaacagcattattccagaagacaccttcttccccagcccagaaagttcctgtgatgtcaagctggtcgagaaaagctttgaaacagatacgaacctaaactttcaaaacctgtcagtgattgggttccgaatcctcctcctgaaagtggccgggtttaatctgctcatgacgctgcggctgtggtccagctga

SEQ ID NO: 144 - DNA, 23 bp, Artificial Sequence
  Primer
tcaggcagtatctggagtcattg

SEQ ID NO: 145 - DNA, 20 bp, Artificial Sequence
  Primer
gcacctccttcccattcacc

SEQ ID NO: 146 - DNA, 22 bp, Artificial Sequence
  Primer
gcttctgatggctcaaacacag

SEQ ID NO: 147 - DNA, 21 bp, Artificial Sequence
  Primer
atggatacctggctcgtatgc

SEQ ID NO: 148 - DNA, 18 bp, Artificial Sequence
  Primer
atgggctgcaggctcctc

SEQ ID NO: 149 - DNA, 18 bp, Artificial Sequence
  Primer
atgggctgcaggctgctc

SEQ ID NO: 150 - DNA, 19 bp, Artificial Sequence
  Primer
atgggctccaggctgctct

SEQ ID NO: 151 - DNA, 14 bp, Artificial Sequence
  Primer
atgggccccgggct

SEQ ID NO: 152 - DNA, 17 bp, Artificial Sequence
  Primer
atgggccctgggctcct

SEQ ID NO: 153 - DNA, 19 bp, Artificial Sequence
  Primer
atgggacccaggctcctct

SEQ ID NO: 154 - DNA, 20 bp, Artificial Sequence
  Primer
atgagcatcgggctcctgtg

SEQ ID NO: 155 - DNA, 18 bp, Artificial Sequence
  Primer
atgagcctcgggctcctg

SEQ ID NO: 156 - DNA, 21 bp, Artificial Sequence
  Primer
atgagaatcaggctcctgtgc

SEQ ID NO: 157 - DNA, 20 bp, Artificial Sequence
  Primer
atgagcatcggcctcctgtg

SEQ ID NO: 158 - DNA, 20 bp, Artificial Sequence
  Primer
atgagcatcagcctcctgtg

SEQ ID NO: 159 - DNA, 20 bp, Artificial Sequence
  Primer
atgggcacaaggctcctctg

SEQ ID NO: 160 - DNA, 18 bp, Artificial Sequence
  Primer
atgggcaccaggctcctc

SEQ ID NO: 161 - DNA, 21 bp, Artificial Sequence
  Primer
atgggcaccagtctcctatgc

SEQ ID NO: 162 - DNA, 23 bp, Artificial Sequence
  Primer
atgggtaccagtctcctatgctg

SEQ ID NO: 163 - DNA, 18 bp, Artificial Sequence
  Primer
atgggcaccagcctcctc

SEQ ID NO: 164 - DNA, 20 bp, Artificial Sequence
  Primer
atgggcttcaggctcctctg

SEQ ID NO: 165 - DNA, 21 bp, Artificial Sequence
  Primer
atgggcacgaggctcttcttc

SEQ ID NO: 166 - DNA, 21 bp, Artificial Sequence
  Primer
atgggcaccaggctcttcttc

SEQ ID NO: 167 - DNA, 21 bp, Artificial Sequence
  Primer
atgggcacaaggttgttcttc

SEQ ID NO: 168 - DNA, 21 bp, Artificial Sequence
  Primer
atgagcaccaggcttctctgc

SEQ ID NO: 169 - DNA, 20 bp, Artificial Sequence
  Primer
atgggtaccaggctcctctg

SEQ ID NO: 170 - DNA, 22 bp, Artificial Sequence
  Primer
atggactcctggaccttctgct

SEQ ID NO: 171 - DNA, 20 bp, Artificial Sequence
  Primer
atggactcctggaccctctg

SEQ ID NO: 172 - DNA, 18 bp, Artificial Sequence
  Primer
atggccaccaggctcctc

SEQ ID NO: 173 - DNA, 22 bp, Artificial Sequence
  Primer
atgcttagtcctgacctgcctg

SEQ ID NO: 174 - DNA, 22 bp, Artificial Sequence
  Primer
atggtttccaggcttctcagtt

SEQ ID NO: 175 - DNA, 19 bp, Artificial Sequence
  Primer
atgggtcctgggcttctcc

SEQ ID NO: 176 - DNA, 22 bp, Artificial Sequence
  Primer
atgagcccaatattcacctgca

SEQ ID NO: 177 - DNA, 22 bp, Artificial Sequence
  Primer
atggatatctggctcctctgct

SEQ ID NO: 178 - DNA, 23 bp, Artificial Sequence
  Primer
atggacaccagagtactctgctg

SEQ ID NO: 179 - DNA, 20 bp, Artificial Sequence
  Primer
atgagcaaccaggtgctctg

SEQ ID NO: 180 - DNA, 19 bp, Artificial Sequence
  Primer
atgctgctgcttctgctgc

SEQ ID NO: 181 - DNA, 24 bp, Artificial Sequence
  Primer
atgactatcaggctcctctgctac

SEQ ID NO: 182 - DNA, 16 bp, Artificial Sequence
  Primer
atgggcccccagctcc

SEQ ID NO: 183 - DNA, 22 bp, Artificial Sequence
  Primer
atgggaatcaggctcctctgtc

SEQ ID NO: 184 - DNA, 24 bp, Artificial Sequence
  Primer
atgctgagtcttctgctccttctc

SEQ ID NO: 185 - DNA, 20 bp, Artificial Sequence
  Primer
atgctctgctctctccttgc

SEQ ID NO: 186 - DNA, 22 bp, Artificial Sequence
  Primer
tcactctgaagatccggtccac

SEQ ID NO: 187 - DNA, 22 bp, Artificial Sequence
  Primer
cttcacatcaattccctggagc

SEQ ID NO: 188 - DNA, 19 bp, Artificial Sequence
  Primer
cacctgaatgccccaacag

SEQ ID NO: 189 - DNA, 21 bp, Artificial Sequence
  Primer
agtcgcttctcacctgaatgc

SEQ ID NO: 190 - DNA, 24 bp, Artificial Sequence
  Primer
gagatgaatgtgagcaccttggag

SEQ ID NO: 191 - DNA, 24 bp, Artificial Sequence
  Primer
gagatgaatgtgagtgccttggag

SEQ ID NO: 192 - DNA, 22 bp, Artificial Sequence
  Primer
gctctgagctgaatgtgaacgc

SEQ ID NO: 193 - DNA, 22 bp, Artificial Sequence
  Primer
gaagtccccaatggctacaatg

SEQ ID NO: 194 - DNA, 21 bp, Artificial Sequence
  Primer
aggtccctgatggctacaatg

SEQ ID NO: 195 - DNA, 20 bp, Artificial Sequence
  Primer
tggcgtctgctgtaccctct

SEQ ID NO: 196 - DNA, 20 bp, Artificial Sequence
  Primer
acagaggatttcccgctcag

SEQ ID NO: 197 - DNA, 20 bp, Artificial Sequence
  Primer
cccctcaagctggagtcagc

SEQ ID NO: 198 - DNA, 23 bp, Artificial Sequence
  Primer
acacagaggatttcccactcagg

SEQ ID NO: 199 - DNA, 22 bp, Artificial Sequence
  Primer
ttctctgcacagaggtctgagg

SEQ ID NO: 200 - DNA, 20 bp, Artificial Sequence
  Primer
gctgcccagtgatcgcttct

SEQ ID NO: 201 - DNA, 22 bp, Artificial Sequence
  Primer
actctgaagatccagcgcacag

SEQ ID NO: 202 - DNA, 23 bp, Artificial Sequence
  Primer
cgtctccactctgaagatccagc

SEQ ID NO: 203 - DNA, 20 bp, Artificial Sequence
  Primer
ggcctgagggatccatctcc

SEQ ID NO: 204 - DNA, 20 bp, Artificial Sequence
  Primer
ggctgctcagtgatcggttc

SEQ ID NO: 205 - DNA, 22 bp, Artificial Sequence
  Primer
gaacgattctccgcacaacagt

SEQ ID NO: 206 - DNA, 24 bp, Artificial Sequence
  Primer
acaaaggagaagtctcagatggct

SEQ ID NO: 207 - DNA, 22 bp, Artificial Sequence
  Primer
ccctcactctggagtcagctac

SEQ ID NO: 208 - DNA, 21 bp, Artificial Sequence
  Primer
cctcactctggagtccgctac

SEQ ID NO: 209 - DNA, 24 bp, Artificial Sequence
  Primer
gcagagaggctcaaaggagtagac

SEQ ID NO: 210 - DNA, 20 bp, Artificial Sequence
  Primer
atccagccctcagaacccag

SEQ ID NO: 211 - DNA, 25 bp, Artificial Sequence
  Primer
atcattctgaactgaacatgagctc

SEQ ID NO: 212 - DNA, 25 bp, Artificial Sequence
  Primer
tggagggacgtattctactctgaag

SEQ ID NO: 213 - DNA, 24 bp, Artificial Sequence
  Primer
gacacccctgataacttccaatcc

SEQ ID NO: 214 - DNA, 20 bp, Artificial Sequence
  Primer
tgcctcccaaattcaccctg

SEQ ID NO: 215 - DNA, 17 bp, Artificial Sequence
  Primer
catcccgcagagccgag

SEQ ID NO: 216 - DNA, 21 bp, Artificial Sequence
  Primer
gcaggtagtgcgaggagattc

SEQ ID NO: 217 - DNA, 20 bp, Artificial Sequence
  Primer
ctgtgacatcggcccaaaag

SEQ ID NO: 218 - DNA, 20 bp, Artificial Sequence
  Primer
acagtgaccagtgcccatcc

SEQ ID NO: 219 - DNA, 19 bp, Artificial Sequence
  Primer
caatgccccaagaacgcac

SEQ ID NO: 220 - DNA, 21 bp, Artificial Sequence
  Primer
tagagtctgccatccccaacc

SEQ ID NO: 221 - DNA, 21 bp, Artificial Sequence
  Primer
gacggagcattttcccctgac

SEQ ID NO: 222 - DNA, 20 bp, Artificial Sequence
  Primer
gccagcaccaaccagacatc

SEQ ID NO: 223 - DNA, 20 bp, Artificial Sequence
  Primer
ctgatcctggagtcgcccag

SEQ ID NO: 224 - DNA, 20 bp, Artificial Sequence
  Primer
atcagccgcccaaacctaac

SEQ ID NO: 225 - DNA, 24 bp, Artificial Sequence
  Primer
cggcagttcatcctgagttctaag

SEQ ID NO: 226 - DNA, 20 bp, Artificial Sequence
  Primer
cgaccagcttgacatcacag

SEQ ID NO: 227 - DNA, 25 bp, Artificial Sequence
  Primer
gttgctcttgaagtccatagacctc

SEQ ID NO: 228 - DNA, 20 bp, Artificial Sequence
  Primer
cagggtcagggttctggata

SEQ ID NO: 229 - DNA, 22 bp, Artificial Sequence
  Primer
atgtggggagctttccttctct

SEQ ID NO: 230 - DNA, 25 bp, Artificial Sequence
  Primer
atgtggggagttttccttctttatg

SEQ ID NO: 231 - DNA, 21 bp, Artificial Sequence
  Primer
atggctttgcagagcactctg

SEQ ID NO: 232 - DNA, 20 bp, Artificial Sequence
  Primer
atggcctctgcacccatctc

SEQ ID NO: 233 - DNA, 20 bp, Artificial Sequence
  Primer
atgaggcaagtggcgagagt

SEQ ID NO: 234 - DNA, 24 bp, Artificial Sequence
  Primer
atgaagacatttgctggattttcg

SEQ ID NO: 235 - DNA, 22 bp, Artificial Sequence
  Primer
atggagtcattcctgggaggtg

SEQ ID NO: 236 - DNA, 22 bp, Artificial Sequence
  Primer
atggagaagatgcggagacctg

SEQ ID NO: 237 - DNA, 22 bp, Artificial Sequence
  Primer
atgctcctgttgctcataccag

SEQ ID NO: 238 - DNA, 19 bp, Artificial Sequence
  Primer
atgctcctgctgctcgtcc

SEQ ID NO: 239 - DNA, 21 bp, Artificial Sequence
  Primer
atgctcctggagcttatccca

SEQ ID NO: 240 - DNA, 24 bp, Artificial Sequence
  Primer
atgctcttagtggtcattctgctg

SEQ ID NO: 241 - DNA, 23 bp, Artificial Sequence
  Primer
atgaattcttctccaggaccagc

SEQ ID NO: 242 - DNA, 28 bp, Artificial Sequence
  Primer
atgaactattctccaggcttagtatctc

SEQ ID NO: 243 - DNA, 24 bp, Artificial Sequence
  Primer
atgaaaaagcatctgacgaccttc

SEQ ID NO: 244 - DNA, 27 bp, Artificial Sequence
  Primer
atgatatccttgagagttttactggtg

SEQ ID NO: 245 - DNA, 30 bp, Artificial Sequence
  Primer
atgaaatccttgagagttttactagtgatc

SEQ ID NO: 246 - DNA, 28 bp, Artificial Sequence
  Primer
atgatgaaatccttgagagttttactgg

SEQ ID NO: 247 - DNA, 26 bp, Artificial Sequence
  Primer
atgacatccattcgagctgtatttat

SEQ ID NO: 248 - DNA, 19 bp, Artificial Sequence
  Primer
atggcaggcattcgagctt

SEQ ID NO: 249 - DNA, 24 bp, Artificial Sequence
  Primer
atgtcactttctagcctgctgaag

SEQ ID NO: 250 - DNA, 22 bp, Artificial Sequence
  Primer
atgaagcccaccctcatctcag

SEQ ID NO: 251 - DNA, 23 bp, Artificial Sequence
  Primer
atggaaactctcctgggagtgtc

SEQ ID NO: 252 - DNA, 22 bp, Artificial Sequence
  Primer
atgctgtctgcttcctgctcag

SEQ ID NO: 253 - DNA, 19 bp, Artificial Sequence
  Primer
atgctgactgccagcctgt

SEQ ID NO: 254 - DNA, 23 bp, Artificial Sequence
  Primer
atggagaaaatgttggagtgtgc

SEQ ID NO: 255 - DNA, 20 bp, Artificial Sequence
  Primer
atggagaccctcttgggcct

SEQ ID NO: 256 - DNA, 24 bp, Artificial Sequence
  Primer
atgaagaggatattgggagctctg

SEQ ID NO: 257 - DNA, 25 bp, Artificial Sequence
  Primer
atggacaagatcttaggagcatcat

SEQ ID NO: 258 - DNA, 20 bp, Artificial Sequence
  Primer
atgctgttctccagcctgct

SEQ ID NO: 259 - DNA, 22 bp, Artificial Sequence
  Primer
atggagaagaatcctttggcag

SEQ ID NO: 260 - DNA, 25 bp, Artificial Sequence
  Primer
atgctactcatcacatcaatgttgg

SEQ ID NO: 261 - DNA, 23 bp, Artificial Sequence
  Primer
atgaggctggtggcaagagtaac

SEQ ID NO: 262 - DNA, 25 bp, Artificial Sequence
  Primer
atgaagttggtgacaagcattactg

SEQ ID NO: 263 - DNA, 23 bp, Artificial Sequence
  Primer
atggtcctgaaattctccgtgtc

SEQ ID NO: 264 - DNA, 17 bp, Artificial Sequence
  Primer
atggccatgctcctggg

SEQ ID NO: 265 - DNA, 23 bp, Artificial Sequence
  Primer
atggagactctcctgaaagtgct

SEQ ID NO: 266 - DNA, 25 bp, Artificial Sequence
  Primer
atggagactgttctgcaagtactcc

SEQ ID NO: 267 - DNA, 28 bp, Artificial Sequence
  Primer
atgctccttgaacatttattaataatct

SEQ ID NO: 268 - DNA, 25 bp, Artificial Sequence
  Primer
atgatgaagtgtccacaggctttac

SEQ ID NO: 269 - DNA, 23 bp, Artificial Sequence
  Primer
atgacacgagttagcttgctgtg

SEQ ID NO: 270 - DNA, 18 bp, Artificial Sequence
  Primer
atggcatgccctggcttc

SEQ ID NO: 271 - DNA, 27 bp, Artificial Sequence
  Primer
atgaagaagctactagcaatgattctg

SEQ ID NO: 272 - DNA, 28 bp, Artificial Sequence
  Primer
atgaactcctctctggactttctaattc

SEQ ID NO: 273 - DNA, 20 bp, Artificial Sequence
  Primer
atggtgaagatccggcaatt

SEQ ID NO: 274 - DNA, 26 bp, Artificial Sequence
  Primer
tccttagtcgctctgatagttatggt

SEQ ID NO: 275 - DNA, 27 bp, Artificial Sequence
  Primer
tttcttcattccttagtcggtctaaag

SEQ ID NO: 276 - DNA, 22 bp, Artificial Sequence
  Primer
ctcttcatcgctgctcatcctc

SEQ ID NO: 277 - DNA, 20 bp, Artificial Sequence
  Primer
gccaaacctccttccacctg

SEQ ID NO: 278 - DNA, 20 bp, Artificial Sequence
  Primer
cctgccgacagaaagtccag

SEQ ID NO: 279 - DNA, 20 bp, Artificial Sequence
  Primer
cgcattgcagacacccagac

SEQ ID NO: 280 - DNA, 26 bp, Artificial Sequence
  Primer
ttgataccacccttaaacagagtttg

SEQ ID NO: 281 - DNA, 25 bp, Artificial Sequence
  Primer
attactgaagaatggaagcagcttg

SEQ ID NO: 282 - DNA, 25 bp, Artificial Sequence
  Primer
tcctttaatctgaggaaaccctctg

SEQ ID NO: 283 - DNA, 22 bp, Artificial Sequence
  Primer
gtgaaacctccttccacctgac

SEQ ID NO: 284 - DNA, 24 bp, Artificial Sequence
  Primer
aggctttgaggctgaatttaagag

SEQ ID NO: 285 - DNA, 27 bp, Artificial Sequence
  Primer
ggctgaatttaacaagagtcaaacttc

SEQ ID NO: 286 - DNA, 22 bp, Artificial Sequence
  Primer
gagcgaaacctccttctacctg

SEQ ID NO: 287 - DNA, 23 bp, Artificial Sequence
  Primer
aaaccacttctttccacttggag

SEQ ID NO: 288 - DNA, 23 bp, Artificial Sequence
  Primer
caaagcaaagctctctgcacatc

SEQ ID NO: 289 - DNA, 22 bp, Artificial Sequence
  Primer
cagtgattcagccacctacctc

SEQ ID NO: 290 - DNA, 26 bp, Artificial Sequence
  Primer
cgaattgctgttacattgaacaagac

SEQ ID NO: 291 - DNA, 23 bp, Artificial Sequence
  Primer
ttgcagctactcaacctggagac

SEQ ID NO: 292 - DNA, 21 bp, Artificial Sequence
  Primer
atccgccaaccttgtcatctc

SEQ ID NO: 293 - DNA, 21 bp, Artificial Sequence
  Primer
aaggcgagacatctttccacc

SEQ ID NO: 294 - DNA, 26 bp, Artificial Sequence
  Primer
agattaagagtcacgcttgacacttc

SEQ ID NO: 295 - DNA, 26 bp, Artificial Sequence
  Primer
gccagtcctatcaagagtgacagttc

SEQ ID NO: 296 - DNA, 23 bp, Artificial Sequence
  Primer
caacttcaccatcacagcctcac

SEQ ID NO: 297 - DNA, 22 bp, Artificial Sequence
  Primer
cacatcacagcccctaaacctg

SEQ ID NO: 298 - DNA, 22 bp, Artificial Sequence
  Primer
tggaagacttaatgcctcgctg

SEQ ID NO: 299 - DNA, 21 bp, Artificial Sequence
  Primer
tgtcgctacggaacgctacag

SEQ ID NO: 300 - DNA, 25 bp, Artificial Sequence
  Primer
cttcaataaaagtgccaagcagttc

SEQ ID NO: 301 - DNA, 25 bp, Artificial Sequence
  Primer
aaaaagtggtcgctattctgtcaac

SEQ ID NO: 302 - DNA, 24 bp, Artificial Sequence
  Primer
gaagaaaggacgaataagtgccac

SEQ ID NO: 303 - DNA, 22 bp, Artificial Sequence
  Primer
acatcacagccacccagactac

SEQ ID NO: 304 - DNA, 24 bp, Artificial Sequence
  Primer
cacagaagacagaaagtccagcac

SEQ ID NO: 305 - DNA, 23 bp, Artificial Sequence
  Primer
gcaatcgctgaagacagaaagtc

SEQ ID NO: 306 - DNA, 25 bp, Artificial Sequence
  Primer
gaaaggacagttctctccacatcac

SEQ ID NO: 307 - DNA, 22 bp, Artificial Sequence
  Primer
aaaagtgccaagcacctctctc

SEQ ID NO: 308 - DNA, 22 bp, Artificial Sequence
  Primer
gcaaagctccctgtaccttacg

SEQ ID NO: 309 - DNA, 25 bp, Artificial Sequence
  Primer
aaagataactgccaagttggatgag

SEQ ID NO: 310 - DNA, 26 bp, Artificial Sequence
  Primer
cttcctgaatatctcagcatccatac

SEQ ID NO: 311 - DNA, 22 bp, Artificial Sequence
  Primer
gcatcctgaacatcacagccac

SEQ ID NO: 312 - DNA, 25 bp, Artificial Sequence
  Primer
gaatcgtttctctgtgaacttccag

SEQ ID NO: 313 - DNA, 21 bp, Artificial Sequence
  Primer
tctcagcaccctccacatcac

SEQ ID NO: 314 - DNA, 24 bp, Artificial Sequence
  Primer
caggtatcagactcagccgtgtac

SEQ ID NO: 315 - DNA, 25 bp, Artificial Sequence
  Primer
gccacaataaacatacaggaaaagc

SEQ ID NO: 316 - DNA, 48 bp, Artificial Sequence
  Primer
atttcaggtgtcgtgaagcggccgcgccaccatgagcatcggcctcct

SEQ ID NO: 317 - DNA, 48 bp, Artificial Sequence; identical to SEQ ID NO: 316
  Primer

SEQ ID NO: 318 - DNA, 48 bp, Artificial Sequence
  Primer
atttcaggtgtcgtgaagcggccgcgccaccatgctgctgcttctgct

SEQ ID NO: 319 - DNA, 48 bp, Artificial Sequence
  Primer
atttcaggtgtcgtgaagcggccgcgccaccatgagcaaccaggtgct

SEQ ID NO: 320 - DNA, 48 bp, Artificial Sequence
  Primer
atttcaggtgtcgtgaagcggccgcgccaccatgggcccccagctcct

SEQ ID NO: 321 - DNA, 49 bp, Artificial Sequence
  Primer
atttcaggtgtcgtgaagcggccgcgccaccatgggctgcaggctgctc

SEQ ID NO: 322 - DNA, 49 bp, Artificial Sequence; identical to SEQ ID NO: 321
  Primer

SEQ ID NO: 323 - DNA, 48 bp, Artificial Sequence
  Primer
atttcaggtgtcgtgaagcggccgcgccaccatgggccctgggctcct

SEQ ID NO: 324 - DNA, 54 bp, Artificial Sequence
  Primer
atttcaggtgtcgtgaagcggccgcgccaccatggacaccagagtactctgctg

SEQ ID NO: 325 - DNA, 47 bp, Artificial Sequence
  Primer
atttcaggtgtcgtgaagcggccgcgccaccatgggcccccagctcc

SEQ ID NO: 326 - DNA, 48 bp, Artificial Sequence; identical to SEQ ID NO: 323
  Primer

SEQ ID NO: 327 - DNA, 51 bp, Artificial Sequence
  Primer
atttcaggtgtcgtgaagcggccgcgccaccatgggcttcaggctcctctg

SEQ ID NO: 328 - DNA, 49 bp, Artificial Sequence; identical to SEQ ID NO: 321
  Primer

SEQ ID NO: 329 - DNA, 49 bp, Artificial Sequence; identical to SEQ ID NO: 321
  Primer

SEQ ID NO: 330 - DNA, 52 bp, Artificial Sequence
  Primer
atttcaggtgtcgtgaagcggccgcgccaccatggatacctggctcgtatgc

SEQ ID NO: 331 - DNA, 49 bp, Artificial Sequence
  Primer
atttcaggtgtcgtgaagcggccgcgccaccatgggcaccaggctcctc

SEQ ID NO: 332 - DNA, 49 bp, Artificial Sequence; identical to SEQ ID NO: 321
  Primer

SEQ ID NO: 333 - DNA, 49 bp, Artificial Sequence; identical to SEQ ID NO: 331
  Primer

SEQ ID NO: 334 - DNA, 51 bp, Artificial Sequence
  Primer
atttcaggtgtcgtgaagcggccgcgccaccatgagcaaccaggtgctctg

SEQ ID NO: 335 - DNA, 47 bp, Artificial Sequence; identical to SEQ ID NO: 325
  Primer

SEQ ID NO: 336 - DNA, 46 bp, Artificial Sequence
  Primer
atttcaggtgtcgtgaagcggccgcgccaccatggactcctggacc

SEQ ID NO: 337 - DNA, 49 bp, Artificial Sequence; identical to SEQ ID NO: 331
  Primer

SEQ ID NO: 338 - DNA, 81 bp, Artificial Sequence
  Primer
tctccagcctgcttcagcaggctgaagttagtagctccgcttccgctccgtttccgccggaaatcctttctcttgaccatg

SEQ ID NO: 339 - DNA, 71 bp, Artificial Sequence
  Primer
tcagcctgctgaagcaggctggagacgtggaggagaaccctggacctatggaaactctcctgggagtgtct

SEQ ID NO: 340 - DNA, 71 bp, Artificial Sequence; identical to SEQ ID NO: 339
  Primer

SEQ ID NO: 341 - DNA, 71 bp, Artificial Sequence
  Primer
tcagcctgctgaagcaggctggagacgtggaggagaaccctggacctatggagaagaatcctttggcagcc

SEQ ID NO: 342 - DNA, 71 bp, Artificial Sequence
  Primer
tcagcctgctgaagcaggctggagacgtggaggagaaccctggacctatgacatccattcgagctgtattt

SEQ ID NO: 343 - DNA, 71 bp, Artificial Sequence
  Primer
tcagcctgctgaagcaggctggagacgtggaggagaaccctggacctatgatgaaatccttgagagtttta

SEQ ID NO: 344 - DNA, 71 bp, Artificial Sequence
  Primer
tcagcctgctgaagcaggctggagacgtggaggagaaccctggacctatgaagaggatattgggagctctg

SEQ ID NO: 345 - DNA, 71 bp, Artificial Sequence; identical to SEQ ID NO: 344
  Primer

SEQ ID NO: 346 - DNA, 74 bp, Artificial Sequence
  Primer
tcagcctgctgaagcaggctggagacgtggaggagaaccctggacctatgaagaagctactagcaatgattctg

SEQ ID NO: 347 - DNA, 73 bp, Artificial Sequence
  Primer
tcagcctgctgaagcaggctggagacgtggaggagaaccctggacctatgacatccattcgagctgtatttat

SEQ ID NO: 348 - DNA, 73 bp, Artificial Sequence; identical to SEQ ID NO: 347
  Primer

SEQ ID NO: 349 - DNA, 74 bp, Artificial Sequence; identical to SEQ ID NO: 346
  Primer

SEQ ID NO: 350 - DNA, 71 bp, Artificial Sequence; identical to SEQ ID NO: 344
  Primer

SEQ ID NO: 351 - DNA, 71 bp, Artificial Sequence; identical to SEQ ID NO: 344
  Primer

SEQ ID NO: 352 - DNA, 71 bp, Artificial Sequence; identical to SEQ ID NO: 344
  Primer

SEQ ID NO: 353 - DNA, 74 bp, Artificial Sequence; identical to SEQ ID NO: 346
  Primer

SEQ ID NO: 354 - DNA, 66 bp, Artificial Sequence
  Primer
tcagcctgctgaagcaggctggagacgtggaggagaaccctggacctatgctgactgccagcctgt

SEQ ID NO: 355 - DNA, 71 bp, Artificial Sequence; identical to SEQ ID NO: 344
  Primer

SEQ ID NO: 356 - DNA, 67 bp, Artificial Sequence
  Primer
tcagcctgctgaagcaggctggagacgtggaggagaaccctggacctatggagaccctcttgggcct

SEQ ID NO: 357 - DNA, 71 bp, Artificial Sequence
  Primer
tcagcctgctgaagcaggctggagacgtggaggagaaccctggacctatgtcactttctagcctgctgaag

SEQ ID NO: 358 - DNA, 66 bp, Artificial Sequence
  Primer
tcagcctgctgaagcaggctggagacgtggaggagaaccctggacctatggcaggcattcgagctt

SEQ ID NO: 359 - DNA, 73 bp, Artificial Sequence; identical to SEQ ID NO: 347
  Primer

SEQ ID NO: 360 - DNA, 74 bp, Artificial Sequence; identical to SEQ ID NO: 346
  Primer

SEQ ID NO: 361 - DNA, 45 bp, Artificial Sequence
  Primer
agggatcctctagactcgagctagctcagctggaccacagccgca

SEQ ID NO: 362 - DNA, 25 bp, Artificial Sequence
  Primer
caccgtctctcagctggtacacggc

SEQ ID NO: 363 - DNA, 25 bp, Artificial Sequence
  Primer
aaacgccgtgtaccagctgagagac

SEQ ID NO: 364 - DNA, 25 bp, Artificial Sequence
  Primer
caccgggctcaaacacagcgacctc

SEQ ID NO: 365 - DNA, 25 bp, Artificial Sequence
  Primer
aaacgaggtcgctgtgtttgagccc

SEQ ID NO: 366 - DNA, 21 bp, Artificial Sequence
  Primer
atggcctccctgctcttcttc